European Patent Application EP 4 310 097 A2, published January 24, 2024. Title: CHIMERIC ANTIGEN RECEPTORS TARGETING B-CELL MATURATION ANTIGEN AND USES THEREOF. Applicant: MEMORIAL SLOAN-KETTERING CANCER CENTER. Application EP JA89520P.EPP. The sequence listing filed with the application follows.

SEQUENCE LISTING (280 sequences)

SEQ ID NO: 1 - protein, 123 aa, synthetic construct
  REGION 1..123: note = Description of Artificial Sequence: Synthetic polypeptide
QVQLQQSGPGLVKPSQTLSLTCAISGDSVSSNSAAWNWIRQSPSRGLEWLGRTYYRSKWYNDYAVSVKSRITINPDTSKNQFSLQLNSVTPEDTAVYYCARQGYSYYGYSDVWGQGTLVTVSS

SEQ ID NO: 2 - protein, 111 aa, synthetic construct
  REGION 1..111: note = Description of Artificial Sequence: Synthetic polypeptide
QSVLTQPPSVSVAPRQRVTISCSGSSSNIGHNDVSWYQHLPGKAPRLLIYFDDLLPSGVSDRFSASKSGTSASLAISGLQSEDEADYYCAAWDGSLNAFVFGTGTKVTVLG

SEQ ID NO: 3 - DNA, 369 bp, synthetic construct
  misc_feature 1..369: note = Description of Artificial Sequence: Synthetic polynucleotide
  source 1..369: mol_type = other DNA
caggtacagctgcagcagtcaggtccaggactggtgaagccctcgcagaccctctcactcacctgtgccatctccggggacagtgtctctagcaacagtgctgcttggaactggatcaggcagtccccatcgagaggccttgagtggctgggaaggacatactacaggtccaagtggtataatgattatgcagtatctgtgaaaagtcgaataaccatcaacccagacacatccaagaaccagttctccctgcagctgaactctgtgactcccgaggacacggctgtgtattactgtgcgcgccagggttactcttactacggttactctgatgtttggggtcaaggtactctggtgaccgtctcctca

SEQ ID NO: 4 - DNA, 333 bp, synthetic construct
  misc_feature 1..333: note = Description of Artificial Sequence: Synthetic polynucleotide
  source 1..333: mol_type = other DNA
cagtctgtgctgactcagccaccctcggtgtctgtagcccccaggcagagggtcaccatctcgtgttctggaagcagctccaacatcggacataatgatgtaagctggtaccagcatctcccagggaaggctcccagactcctcatctattttgatgacctgctgccgtcaggggtctctgaccgattctctgcctccaagtctggcacctcagcctccctggccatcagtgggctccagtctgaggatgaggctgattattactgtgcagcatgggatggcagcctgaatgcctttgtcttcggaactgggaccaaggtcaccgtcctaggt

SEQ ID NO: 5 - protein, 123 aa, synthetic construct
  REGION 1..123: note = Description of Artificial Sequence: Synthetic polypeptide
QVQLQQSGPGLVKPSQTLSLTCAISGDSVSSNSAAWNWIRQSPSRGLEWLGRTYYRSKWYNDYAVSVKSRITINPDTSKNQFSLQLNSVTPEDTAVYYCARYGFSGSRFYDTWGQGTLVTVSS

SEQ ID NO: 6 - protein, 111 aa, synthetic construct
  REGION 1..111: note = Description of Artificial Sequence: Synthetic polypeptide
QPVLTQPPSVSEAPRQRVTISCSGSSSNIGNNAVNWYQQLPGKAPKLLIYFDDLLSSGVSDRFSGSKSGTSASLAISGLQSEDEADYYCAAWDDSLNGYVFGTGTKVTVLG

SEQ ID NO: 7 - DNA, 369 bp, synthetic construct
  misc_feature 1..369: note = Description of Artificial Sequence: Synthetic polynucleotide
  source 1..369: mol_type = other DNA
caggtacagctgcagcagtcaggtccaggactggtgaagccctcgcagaccctctcactcacctgtgccatctccggggacagtgtctctagcaacagtgctgcttggaactggatcaggcagtccccatcgagaggccttgagtggctgggaaggacatactacaggtccaagtggtataatgattatgcagtatctgtgaaaagtcgaataaccatcaacccagacacatccaagaaccagttctccctgcagctgaactctgtgactcccgaggacacggctgtgtattactgtgcgcgctacggtttctctggttctcgtttctacgatacttggggtcaaggtactctggtgaccgtctcctca

SEQ ID NO: 8 - DNA, 333 bp, synthetic construct
  misc_feature 1..333: note = Description of Artificial Sequence: Synthetic polynucleotide
  source 1..333: mol_type = other DNA
cagcctgtgctgactcagccaccctcggtgtctgaagcccccaggcagagggtcaccatctcctgttctggaagcagctccaacatcggaaataatgctgtaaactggtaccagcagctcccaggaaaggctcccaaactcctcatctattttgatgatctgctgtcctcaggggtctctgaccgattctctggctccaagtctggcacctcagcctccctggccatcagtgggctccagtctgaagatgaggctgattattactgtgcagcatgggatgacagcctgaatggttatgtcttcggaactgggaccaaggtcaccgtcctaggt

SEQ ID NO: 9 - protein, 122 aa, synthetic construct
  REGION 1..122: note = Description of Artificial Sequence: Synthetic polypeptide
EVQLVQSGAEVKKPGSSVKVSCKASGGTFSSYAISWVRQAPGQGLEWMGRIIPILGIANYAQKFQGRVTMTEDTSTDTAYMELSSLRSEDTAVYYCARSGYSKSIVSYMDYWGQGTLVTVSS

SEQ ID NO: 10 - protein, 111 aa, synthetic construct
  REGION 1..111: note = Description of Artificial Sequence: Synthetic polypeptide
LPVLTQPPSTSGTPGQRVTVSCSGSSSNIGSNVVFWYQQLPGTAPKLVIYRNNQRPSGVPDRFSVSKSGTSASLAISGLRSEDEADYYCAAWDDSLSGYVFGTGTKVTVLG

SEQ ID NO: 11 - DNA, 366 bp, synthetic construct
  misc_feature 1..366: note = Description of Artificial Sequence: Synthetic polynucleotide
  source 1..366: mol_type = other DNA
gaggtccagctggtgcagtctggagctgaggtgaagaagcctgggtcctcggtgaaggtctcctgcaaggcttctggaggcaccttcagcagctatgctatcagctgggtgcgacaggcccctggacaagggcttgagtggatgggaaggatcatccctatccttggtatagcaaactacgcacagaagttccagggcagagtcaccatgaccgaggacacatctacagacacagcctacatggagctgagcagcctgagatctgaggacacggccgtgtattactgtgcgcgctctggttactctaaatctatcgtttcttacatggattactggggtcaaggtactctggtgaccgtctcctca

SEQ ID NO: 12 - DNA, 333 bp, synthetic construct
  misc_feature 1..333: note = Description of Artificial Sequence: Synthetic polynucleotide
  source 1..333: mol_type = other DNA
ctgcctgtgctgactcagcccccctccacgtctgggacccccgggcagagggtcaccgtctcttgttctggaagcagctccaacatcggaagtaatgttgtattctggtaccagcagctcccaggcacggcccccaaacttgtcatctataggaataatcaacggccctcaggggtccctgaccgattctctgtctccaagtctggcacctcagcctccctggccatcagtgggctccggtccgaggacgaggctgattattattgtgcagcttgggatgacagcctgagtggttatgtcttcggaactgggaccaaggtcaccgtcctaggt

SEQ ID NO: 13 - protein, 118 aa, synthetic construct
  REGION 1..118: note = Description of Artificial Sequence: Synthetic polypeptide
EVQLVQSGAEVKKPGASVKVSCKASGYTFTSYYMHWVRQAPGQGLEWMGIINPSGGSTSYAQKFQGRVTMTRDTSTSTVYMELSSLRSEDTAVYYCARSQWGGVLDYWGQGTLVTVSS

SEQ ID NO: 14 - protein, 112 aa, synthetic construct
  REGION 1..112: note = Description of Artificial Sequence: Synthetic polypeptide
QSVVTQPPSVSGAPGQRVTISCSGSSSNIGARYDVQWYQQLPGTAPKLLIFGNNNRPSGVPDRFSGSKSGTSASLAITGLQAEDEADYYCQSYDSSLSASVFGGGTKLTVLG

SEQ ID NO: 15 - DNA, 354 bp, synthetic construct
  misc_feature 1..354: note = Description of Artificial Sequence: Synthetic polynucleotide
  source 1..354: mol_type = other DNA
gaggtccagctggtacagtctggggctgaggtgaagaagcctggggcctcagtgaaggtttcctgcaaggcatctggatacaccttcaccagctactatatgcactgggtgcgacaggcccctggacaagggcttgagtggatgggaataatcaaccctagtggtggtagcacaagctacgcacagaagttccagggcagagtcaccatgaccagggacacgtccacgagcacagtctacatggagctgagcagcctgagatctgaggacacggccgtgtattactgtgcgcgctctcagtggggtggtgttctggattactggggtcaaggtactctggtgaccgtctcctca

SEQ ID NO: 16 - DNA, 336 bp, synthetic construct
  misc_feature 1..336: note = Description of Artificial Sequence: Synthetic polynucleotide
  source 1..336: mol_type = other DNA
cagtctgtcgtgacgcagccgccctcagtgtctggggccccagggcagagggtcaccatctcctgcagtgggagcagctccaacatcggggcacgttatgatgttcagtggtaccagcagcttccaggaacagcccccaaactcctcatctttggtaacaacaatcggccctcaggggtccctgaccgattctctggctccaagtctggcacgtcagcctccctggccatcactgggctccaggctgaggatgaggctgattattactgccagtcctatgacagcagcctgagtgcttcggtgttcggcggagggaccaagctgaccgtcctaggt

SEQ ID NO: 17 - protein, 123 aa, synthetic construct
  REGION 1..123: note = Description of Artificial Sequence: Synthetic polypeptide
QVQLVESGAEVKKPGSSVKVSCKASGGTFSSYAISWVRQAPGQGLEWMGRIIPILGIANYAQKFQGRVTITADESTSTAYMELSSLRSEDTAVYYCARTGYESWGSYEVIDRWGQGTLVTVSS

SEQ ID NO: 18 - protein, 111 aa, synthetic construct
  REGION 1..111: note = Description of Artificial Sequence: Synthetic polypeptide
QAVLTQPPSASGTPGQRVTISCSGSSSNIGSNTVNWYRQLPGTAPKLLIYSNNQRPSGVPDRFSGSKSGTSASLAISGLQSEDEADYYCAAWDDSLNGVVFGGGTKLTVLG

SEQ ID NO: 19 - DNA, 369 bp, synthetic construct
  misc_feature 1..369: note = Description of Artificial Sequence: Synthetic polynucleotide
  source 1..369: mol_type = other DNA
caggtgcagctggtggagtctggggctgaggtgaagaagcctgggtcctcggtgaaggtctcctgcaaggcttctggaggcaccttcagcagctatgctatcagctgggtgcgacaggcccctggacaagggcttgagtggatgggaaggatcatccctatccttggtatagcaaactacgcacagaagttccagggcagagtcacgattaccgcggacgaatccacgagcacagcctacatggagctgagcagcctgagatctgaggacacggccgtatattactgtgcgcgcactggttacgaatcttggggttcttacgaagttatcgatcgttggggtcaaggtactctggtgaccgtctcctca

SEQ ID NO: 20 - DNA, 333 bp, synthetic construct
  misc_feature 1..333: note = Description of Artificial Sequence: Synthetic polynucleotide
  source 1..333: mol_type = other DNA
caggctgtgctgactcagccaccctcagcgtctgggacccccgggcagagggtcaccatctcttgttctggaagcagctccaacatcggaagtaatactgtaaactggtaccggcagctcccaggaacggcccccaaactcctcatctatagtaataatcagcggccctcaggggtccctgaccgattctctggctccaagtctggcacctcagcctccctggccatcagtgggctccagtctgaggatgaggctgattattactgtgcagcatgggatgacagcctgaatggtgtggtattcggcggagggaccaagctgaccgtcctaggt

SEQ ID NO: 21 - protein, 121 aa, synthetic construct
  REGION 1..121: note = Description of Artificial Sequence: Synthetic polypeptide
QVQLVQSGAEVKKPGSSVKVSCKASGGTFSSYAISWVRQAPGQGLEWMGRIIPILGIANYAQKFQGRVTITADKSTSTAYMELSSLRSEDTAVYYCARGGYYSHDMWSEDWGQGTLVTVSS

SEQ ID NO: 22 - protein, 112 aa, synthetic construct
  REGION 1..112: note = Description of Artificial Sequence: Synthetic polypeptide
LPVLTQPPSASGTPGQRVTISCSGRSSNIGSNSVNWYRQLPGAAPKLLIYSNNQRPPGVPVRFSGSKSGTSASLAISGLQSEDEATYYCATWDDNLNVHYVFGTGTKVTVLG

SEQ ID NO: 23 - DNA, 363 bp, synthetic construct
  misc_feature 1..363: note = Description of Artificial Sequence: Synthetic polynucleotide
  source 1..363: mol_type = other DNA
caggtgcagctggtgcagtctggggctgaggtgaagaagcctgggtcctcggtgaaggtctcctgcaaggcttctggaggcaccttcagcagctatgctatcagctgggtgcgacaggcccctggacaagggcttgagtggatgggaaggatcatccctatccttggtatagcaaactacgcacagaagttccagggcagagtcacgattaccgcggacaaatccacgagcacagcctacatggagctgagcagcctgagatctgaggacacggccgtgtattactgtgcgcgcggtggttactactctcatgacatgtggtctgaagattggggtcaaggtactctggtgaccgtctcctca

SEQ ID NO: 24 - DNA, 336 bp, synthetic construct
  misc_feature 1..336: note = Description of Artificial Sequence: Synthetic polynucleotide
  source 1..336: mol_type = other DNA
ctgcctgtgctgactcagccaccctcagcgtctgggacccccgggcagagggtcaccatctcttgttctggacgcagttccaacatcgggagtaattctgttaactggtatcgacaactcccaggagcggcccccaaactcctcatctatagtaataatcagcggcccccaggggtccctgtgcgattctctggctccaagtctggcacctcagcctccctggccatcagtgggctccagtctgaagatgaggccacttattactgtgcaacatgggatgacaatctgaatgttcactatgtcttcggaactgggaccaaggtcaccgtcctaggt

SEQ ID NO: 25 - protein, 125 aa, synthetic construct
  REGION 1..125: note = Description of Artificial Sequence: Synthetic polypeptide
QVQLQESGPGLVKPSGTLSLTCGVSGGSISNSNWWSWVRQPPGKGLEWIGEIYHSGSTKYNPSLRSRVTISVDKSKNQFSLKLSSVTAADTAVYYCARRDNWKTPTTKIDGFDIWGQGTMVTVSS

SEQ ID NO: 26 - protein, 117 aa, synthetic construct
  REGION 1..117: note = Description of Artificial Sequence: Synthetic polypeptide
QPVLTQPPSASASLGASVTLTCTLSSGYSNYKVDWYQQRPGKGPRFVMRVGTGGIVGSKGDGIPDRFSVLGSGLNRYLTIKNIQEEDEGDYHCGADHGSGSNFVYVFGTGTKVTVLG

SEQ ID NO: 27 - DNA, 375 bp, synthetic construct
  misc_feature 1..375: note = Description of Artificial Sequence: Synthetic polynucleotide
  source 1..375: mol_type = other DNA
caggtgcagctgcaggagtcgggcccaggactggtgaagccttcggggaccctgtccctcacctgcggtgtctctggtggctccatcagcaatagtaactggtggagttgggtccgccagccccccgggaaggggctggagtggattggggaaatctatcatagtgggagcaccaagtacaacccgtccctcaggagtcgagtcaccatatcagtagacaagtccaagaaccagttctccctaaaattgagctctgtgaccgccgcggacacggccgtatattactgtgcgagacgagataactggaagacccccactaccaaaattgatggttttgatatctggggccaagggacaatggtcaccgtctcttca

SEQ ID NO: 28 - DNA, 351 bp, synthetic construct
  misc_feature 1..351: note = Description of Artificial Sequence: Synthetic polynucleotide
  source 1..351: mol_type = other DNA
cagcctgtgctgactcagccaccttctgcatcagcctccctgggagcctcggtcacactcacctgcaccctgagcagcggctacagtaattataaagtggactggtaccagcagagaccagggaagggcccccggtttgtgatgcgagtgggcactggtgggattgtgggatccaagggggatggcatccctgatcgcttctcagtcttgggctcaggcctgaatcggtacctgaccatcaagaacatccaggaagaagatgagggtgactatcactgtggggcagaccatggcagtgggagcaacttcgtgtatgtcttcggaactgggaccaaggtcaccgtcctaggt

SEQ ID NO: 29 - protein, 118 aa, synthetic construct
  REGION 1..118: note = Description of Artificial Sequence: Synthetic polypeptide
QVQLVQSGAEVKKPGASVKVSCKASGYTFTGYYMHWVRQAPGQGLEWMGWINPNSGGTNYAQKFQGRVTMTRDTSISTAYMELSRLRSDDTAVYYCARSQWGSSWDYWGQGTLVTVSS

SEQ ID NO: 30 - protein, 108 aa, synthetic construct
  REGION 1..108: note = Description of Artificial Sequence: Synthetic polypeptide
DIQLTQSPSSLSASVGDRVTITCRASQSISSYLNWYQQKPGKAPKLLIYAASSLQSGVPSRFSGSGSGTDFTLTISSLQPEDFATYYCQQSYSTPPTFGQGTKVEIKR

SEQ ID NO: 31 - DNA, 354 bp, synthetic construct
  misc_feature 1..354: note = Description of Artificial Sequence: Synthetic polynucleotide
  source 1..354: mol_type = other DNA
caggtccagctggtacagtctggggctgaggtgaagaagcctggggcctcagtgaaggtctcctgcaaggcttctggatacaccttcaccggctactatatgcactgggtgcgacaggcccctggacaagggcttgagtggatgggatggatcaaccctaacagtggtggcacaaactatgcacagaagtttcagggcagggtcaccatgaccagggacacgtccatcagcacagcctacatggagctgagcaggctgagatctgacgacacggccgtgtattactgtgcgcgctctcagtggggttcttcttgggattactggggtcaaggtactctggtgaccgtctcctca

SEQ ID NO: 32 - DNA, 324 bp, synthetic construct
  misc_feature 1..324: note = Description of Artificial Sequence: Synthetic polynucleotide
  source 1..324: mol_type = other DNA
gacatccagttgacccagtctccatcctccctgtctgcatctgtaggagacagagtcaccatcacttgccgggcaagtcagagcattagcagctatttaaattggtatcagcagaaaccagggaaagcccctaagctcctgatctatgctgcatccagtttgcaaagtggggtcccatcaaggttcagtggcagtggatctgggacagatttcactctcaccatcagcagtctgcaacctgaagattttgcaacttactactgtcaacagagttacagtacccctccgacgttcggccaagggaccaaggtggagatcaaacgt

SEQ ID NO: 33 - protein, 119 aa, synthetic construct
  REGION 1..119: note = Description of Artificial Sequence: Synthetic polypeptide
EVQLVESGAEVKKPGASVKVSCKASGYTFTGYYMHWVRQAPGQGLEWMGWINPNSGGTNYAQKFQGRVTMTRDTSISTAYMELSRLRSDDTAVYYCARSSYHLYGYDSWGQGTLVTVSS

SEQ ID NO: 34 - protein, 117 aa, synthetic construct
  REGION 1..117: note = Description of Artificial Sequence: Synthetic polypeptide
QPVLTQPPSASASLGASVTLTCTLSNDYTNYKVDWYQQRPGKGPRFVMRVGPGGIVGSKGDGIPDRFSVLGSGLNRYLTIKNIQEEDESDYHCGADHGTGSNFVYVFGGGTKLTVLG

SEQ ID NO: 35 - DNA, 357 bp, synthetic construct
  misc_feature 1..357: note = Description of Artificial Sequence: Synthetic polynucleotide
  source 1..357: mol_type = other DNA
gaggtgcagctggtggagtccggggctgaggtgaagaagcctggggcctcagtgaaggtctcctgcaaggcttctggatacaccttcaccggctactatatgcactgggtgcgacaggcccctggacaagggcttgagtggatgggatggatcaaccctaacagtggtggcacaaactatgcacagaagtttcagggcagggtcaccatgaccagggacacgtccatcagcacagcctacatggagctgagcaggctgagatctgacgacacggccgtatattactgtgcgcgctcttcttaccatctgtacggttacgattcttggggtcaaggtactctggtgaccgtctcctca

SEQ ID NO: 36 - DNA, 351 bp, synthetic construct
  misc_feature 1..351: note = Description of Artificial Sequence: Synthetic polynucleotide
  source 1..351: mol_type = other DNA
cagcctgtgctgactcagccaccttctgcatcagcctccctgggagcctcggtcactctcacctgcaccctgagcaacgactacactaattataaagtggactggtaccagcagagaccagggaagggcccccggtttgtgatgcgagtgggccctggtgggattgtgggatccaagggggatggcatccctgatcgcttctcagtcttgggctcaggcctgaatcgatacctgaccatcaagaacatccaggaggaggatgagagtgactaccactgtggggcggaccatggcaccgggagcaacttcgtgtacgtgttcggcggagggaccaagctgaccgtcctaggt

SEQ ID NO: 37 - protein, 120 aa, synthetic construct
  REGION 1..120: note = Description of Artificial Sequence: Synthetic polypeptide
QVQLVQSGAEVKKPGSSVKVSCKASGGTFSSYAISWVRQAPGQGLEWMGGIIPIFSTANYAQKFQGRVTMTTDTSTSTAYMELRSLRSDDTAVYYCARQPWTWYSPYDQWGQGTLVTVSS

SEQ ID NO: 38 - protein, 117 aa, synthetic construct
  REGION 1..117: note = Description of Artificial Sequence: Synthetic polypeptide
QPVLTQPPSASASLGASVTLTCTLSSGYSNYKVDWYQQRPGKGPRFLMRVDTGGIVGSKGDGIPDRFSVSGSGLNRYLTIKNIQEEDESDYHCGADHGSGSNFVWVFGGGTKLTVLG

SEQ ID NO: 39 - DNA, 360 bp, synthetic construct
  misc_feature 1..360: note = Description of Artificial Sequence: Synthetic polynucleotide
  source 1..360: mol_type = other DNA
caggtgcagctggtgcagtctggggctgaggtgaagaagcctgggtcctcggtgaaggtctcctgcaaggcttctggaggcaccttcagcagctatgctatcagctgggtgcgacaggcccctggacaagggcttgagtggatgggagggatcatccctatctttagtacagcaaactacgcacagaagttccagggcagagtcaccatgaccacagacacatccacgagcacagcctacatggagctgaggagcctgagatctgacgacacggccgtgtattactgtgcgcgccagccgtggacttggtactctccgtacgatcagtggggtcaaggtactctggtgaccgtctcctca

SEQ ID NO: 40 - DNA, 351 bp, synthetic construct
  misc_feature 1..351: note = Description of Artificial Sequence: Synthetic polynucleotide
  source 1..351: mol_type = other DNA
cagcctgtgctgactcagccaccttctgcatcagcctccctgggagcctcggtcacactcacctgcaccctgagcagcggctacagtaattataaagtggactggtatcaacagagaccagggaagggcccccggtttctgatgcgagtagacaccggtgggattgtgggatccaagggggatggcatccctgatcgcttctcagtctcgggctcaggtctgaatcggtacctgaccatcaagaacattcaggaagaggatgagagtgactaccactgtggggcagaccatggcagtgggagcaacttcgtgtgggtgttcggcggagggaccaagctgaccgtcctaggt

SEQ ID NO: 41 - protein, 117 aa, synthetic construct
  REGION 1..117: note = Description of Artificial Sequence: Synthetic polypeptide
EVQLVETGGGLVQPGGSLRLSCAASGFTFSTYAMTWVRQAPGKGLEWVSAITPGGDRTYYADSVKGRFTISRDNSRNTLYLQMNSLRAEDTAVYYCARYYGYMIDMWGQGTLVTVSS

SEQ ID NO: 42 - protein, 113 aa, synthetic construct
  REGION 1..113: note = Description of Artificial Sequence: Synthetic polypeptide
DVVMTQSPLSLPVTPGEPASISCRSSQSLLHSNGYNYLDWYLQKPGQSPQLLIYLGSNRASGVPDRFSGSGSGTDFTLKISRVEAEDVGVYYCMQALQTPLTFGGGTKVEIKR

SEQ ID NO: 43 - DNA, 351 bp, synthetic construct
  misc_feature 1..351: note = Description of Artificial Sequence: Synthetic polynucleotide
  source 1..351: mol_type = other DNA
gaggtgcagctggtggagactgggggaggcctggtacagcctggggggtccctgagactctcctgtgctgcctctggattcacctttagcacctatgccatgacctgggtccgccaggctccagggaaggggctggagtgggtctcagctattactcctggtggtgatcgcacatactacgcagactccgtgaagggccgtttcactatctccagagacaattccaggaacacgctgtatctgcaaatgaacagcctgagagccgaggacacggccgtatattactgtgcgcgctactacggttacatgatcgatatgtggggtcaaggtactctggtgaccgtctcctca

SEQ ID NO: 44 - DNA, 339 bp, synthetic construct
  misc_feature 1..339: note = Description of Artificial Sequence: Synthetic polynucleotide
  source 1..339: mol_type = other DNA
gatgttgtgatgactcagtctccactctccctgcccgtcacccctggagagccggcctccatctcctgcaggtctagtcagagcctcctgcatagtaatggatacaactatttggattggtacctgcagaagccagggcagtctccacagctcctgatctatttgggttctaatcgggcctccggggtccctgacaggttcagtggcagtggatcaggcacagattttacactgaaaatcagcagagtggaggctgaggatgttggggtttattactgcatgcaagctctacaaactcctctcactttcggcggagggaccaaggtggaaatcaaacgt

SEQ ID NO: 45 - protein, 118 aa, synthetic construct
  REGION 1..118: note = Description of Artificial Sequence: Synthetic polypeptide
QMQLVQSGAEVKKPGASVKVSCKASGYTFTGYYVHWLRQAPGQGLEWMGWINPNSGGTNNAQEFQGRITMTRDTSINTAYMELSRLRSDDTAVYYCARSQWGGTYDYWGQGTLVTVSS

SEQ ID NO: 46 - protein, 111 aa, synthetic construct
  REGION 1..111: note = Description of Artificial Sequence: Synthetic polypeptide
SYVLTQPPSASGTPGQRVTISCSGSSSNIGSNTVNWYQQVPGTAPKLLIYSNNQRPSGVPDRFSGSKSGASASLAISWLQSEDEADYYCAAWDDSLNGWVFGGGTKLTVLG

SEQ ID NO: 47 - DNA, 354 bp, synthetic construct
  misc_feature 1..354: note = Description of Artificial Sequence: Synthetic polynucleotide
  source 1..354: mol_type = other DNA
cagatgcagctggtgcagtctggggctgaggtgaagaagcctggggcctcagtgaaggtctcctgcaaggcttctggatacaccttcaccggctattatgtacactggttgcgacaggcccctggacaagggcttgagtggatgggttggatcaaccctaacagtggcggcacaaacaatgcacaggagtttcaaggcaggatcaccatgaccagggacacgtccatcaacacagcctacatggagctgagcaggctgagatctgacgacacggccgtgtattactgtgcgcgctctcagtggggtggtacttacgattactggggtcaaggtactctggtgaccgtctcctca

SEQ ID NO: 48 - DNA, 333 bp, synthetic construct
  misc_feature 1..333: note = Description of Artificial Sequence: Synthetic polynucleotide
  source 1..333: mol_type = other DNA
tcctatgtgctgactcagccaccctcagcgtctgggacccccgggcagagggtcaccatctcttgttctggaagcagctccaacatcggaagtaatactgtaaactggtaccagcaggtcccaggaacggcccccaaactcctcatctatagtaataatcagcggccctcaggggtccctgaccgattctctggctccaagtctggcgcctcagcctccctggccatcagttggctccagtctgaggatgaggctgattattactgtgcagcatgggatgacagcctgaatggttgggtgttcggcggagggaccaagctgaccgtcctaggt

SEQ ID NO: 49 - protein, 117 aa, synthetic construct
  REGION 1..117: note = Description of Artificial Sequence: Synthetic polypeptide
EVQLVQSGAEVKKPGESLKISCKGSGYDFTTYWIGWVRQMPGKGLEWMGIIYPGDSDTRYSPSVRGRVTISADKSINTAYLQWSSLEASDTAMYYCARMWTFSQDGWGQGTLVTVSS

SEQ ID NO: 50 - protein, 111 aa, synthetic construct
  REGION 1..111: note = Description of Artificial Sequence: Synthetic polypeptide
QAVLTQPPSASGTPGQRVTISCSGSSSNIGSYTVSWYQQLPGTAPKFLIYSNNQRPSGVPDRFSGSKSGTSASLAISGLQSEDEADYYCAAWDDSLNGYVFGTGTKVTVLG

SEQ ID NO: 51 - DNA, 351 bp, synthetic construct
  misc_feature 1..351: note = Description of Artificial Sequence: Synthetic polynucleotide
  source 1..351: mol_type = other DNA
gaggtgcagctggtgcagtctggagcagaggtgaaaaagccgggggagtctctgaagatctcctgtaagggttctggatatgactttaccacctactggatcgggtgggtgcgccagatgcccgggaagggcctggagtggatggggatcatctatcctggtgactctgataccagatacagcccgtccgtccgaggccgggtcaccatctcagccgacaagtccatcaacaccgcctatttgcagtggagtagcctggaggcctccgacaccgccatgtattactgtgcgcgcatgtggactttctctcaggatggttggggtcaaggtactctggtgaccgtctcctca

SEQ ID NO: 52 - DNA, 333 bp, synthetic construct
  misc_feature 1..333: note = Description of Artificial Sequence: Synthetic polynucleotide
  source 1..333: mol_type = other DNA
caggctgtgctgactcagccaccctcagcgtctgggacccccgggcagagggtcaccatctcttgttctggaagcagctccaacatcggaagttatactgtaagctggtaccagcaactcccaggaacggcccccaaattcctcatctattctaataatcagcggccctcaggggtccctgaccgattctctggctccaagtctggcacctcagcctccctggccatcagtgggctccagtctgaggatgaggctgattattactgtgctgcatgggatgacagcctgaatggttatgtcttcggaactgggaccaaggtcaccgtcctaggt

SEQ ID NO: 53 - protein, 118 aa, synthetic construct
  REGION 1..118: note = Description of Artificial Sequence: Synthetic polypeptide
EVQLVQSGAEMKKPGASLKLSCKASGYTFIDYYVYWMRQAPGQGLESMGWINPNSGGTNYAQKFQGRVTMTRDTSISTAYMELSRLRSDDTAMYYCARSQRDGYMDYWGQGTLVTVSS

SEQ ID NO: 54 - protein, 105 aa, synthetic construct
  REGION 1..105: note = Description of Artificial Sequence: Synthetic polypeptide
QSALTQPASVSASPGQSIAISCTGTSSDVGWYQQHPGKAPKLMIYEDSKRPSGVSNRFSGSKSGNTASLTISGLQAEDEADYYCSSNTRSSTLVFGGGTKLTVLG

SEQ ID NO: 55 - DNA, 354 bp, synthetic construct
  misc_feature 1..354: note = Description of Artificial Sequence: Synthetic polynucleotide
  source 1..354: mol_type = other DNA
gaagtgcagctggtgcagtctggggctgagatgaagaagcctggggcctcactgaagctctcctgcaaggcttctggatacaccttcatcgactactatgtatactggatgcgacaggcccctggacaagggcttgagtccatgggatggatcaaccctaacagtggtggcacaaactatgcacagaagtttcagggcagggtcaccatgaccagggacacgtccatcagcacagcctacatggagctgagcaggctgagatctgacgacaccgccatgtattactgtgcgcgctcccagcgtgacggttacatggattactggggtcaaggtactctggtgaccgtctcctca

SEQ ID NO: 56 - DNA, 315 bp, synthetic construct
  misc_feature 1..315: note = Description of Artificial Sequence: Synthetic polynucleotide
  source 1..315: mol_type = other DNA
caatctgccctgactcagcctgcctccgtgtctgcgtctcctggacagtcgatcgccatctcctgcactggaaccagcagtgacgttggttggtatcaacagcacccaggcaaagcccccaaactcatgatttatgaggacagtaagcggccctcaggggtttctaatcgcttctctggctccaagtctggcaacacggcctccctgaccatctctgggctccaggctgaggacgaggctgattattactgcagctcaaatacaagaagcagcactttggtgttcggcggagggaccaagctgaccgtcctaggt

SEQ ID NO: 57 - protein, 118 aa, synthetic construct
  REGION 1..118: note = Description of Artificial Sequence: Synthetic polypeptide
QVQLVQSGAEVKKPGASVKVSCKASGYTFTDYYMHWVRQAPGQRLEWMGWINPNSGGTNYAQKFQDRITVTRDTSSNTGYMELTRLRSDDTAVYYCARSPYSGVLDKWGQGTLVTVSS

SEQ ID NO: 58 - protein, 112 aa, synthetic construct
  REGION 1..112: note = Description of Artificial Sequence: Synthetic polypeptide
QSVLTQPPSVSGAPGQRVTISCTGSSSNIGAGFDVHWYQQLPGTAPKLLIYGNSNRPSGVPDRFSGSKSGTSASLAITGLQAEDEADYYCQSYDSSLSGYVFGTGTKVTVLG

SEQ ID NO: 59 - DNA, 354 bp, synthetic construct
  misc_feature 1..354: note = Description of Artificial Sequence: Synthetic polynucleotide
  source 1..354: mol_type = other DNA
caggtccagctggtacagtctggggctgaggtgaagaagcctggggcctcagtgaaggtctcctgcaaggcttctggatacaccttcaccgactactatatgcactgggtgcgacaggcccctggacaacggcttgagtggatgggatggatcaaccctaacagtggtggcacaaactatgcacagaagtttcaggacaggatcaccgtgaccagggacacctccagcaacacaggctacatggagctgaccaggctgagatctgacgacacggccgtgtattactgtgcgcgctctccgtactctggtgttctggataaatggggtcaaggtactctggtgaccgtctcctca

SEQ ID NO: 60 - DNA, 336 bp, synthetic construct
  misc_feature 1..336: note = Description of Artificial Sequence: Synthetic polynucleotide
  source 1..336: mol_type = other DNA
cagtctgtgctgacgcagccgccctcagtgtctggggccccagggcagagggtcaccatctcctgcactgggagcagctccaacatcggggcaggttttgatgtacactggtaccagcagcttccaggaacagcccccaaactcctcatctatggtaacagcaatcggccctcaggggtccctgaccgattctctggctccaagtctggcacctcagcctccctggccatcactgggctccaggctgaggatgaggctgattattactgccagtcctatgacagcagcctgagtggttatgtcttcggaactgggaccaaggtcaccgtcctaggt

SEQ ID NO: 61 - protein, 120 aa, synthetic construct
  REGION 1..120: note = Description of Artificial Sequence: Synthetic polypeptide
QVQLVQSGAEVKKPGSSVKVSCKASGGTFSSYAISWVRQAPGQGLEWMGRIIPILGTANYAQKFQGRVTITADESTSTAYMELSSLRSEDTAVYYCARSGYGSYRWEDSWGQGTLVTVSS

SEQ ID NO: 62 - protein, 112 aa, synthetic construct
  REGION 1..112: note = Description of Artificial Sequence: Synthetic polypeptide
QAVLTQPPSASGTPGQRVTISCSGSSSNIGSNYVFWYQQLPGTAPKLLIYSNNQRPSGVPDRFSGSKSGTSASLAISGLRSEDEADYYCAAWDDSLSASYVFGTGTKVTVLG

SEQ ID NO: 63 - DNA, 360 bp, synthetic construct
  misc_feature 1..360: note = Description of Artificial Sequence: Synthetic polynucleotide
  source 1..360: mol_type = other DNA
caggtgcagctggtgcagtctggggctgaggtgaagaagcctgggtcctcggtgaaggtctcctgcaaggcttctggaggcaccttcagcagctatgctatcagctgggtgcgacaggcccctggacaagggcttgagtggatgggaaggatcatccctatccttggtacagcaaactacgcacagaagttccagggcagagtcacgattaccgcggacgaatccacgagcacagcctacatggagctgagcagcctgagatctgaggacacggccgtgtattactgtgcgcgctctggttacggttcttaccgttgggaagattcttggggtcaaggtactctggtgaccgtctcctca

SEQ ID NO: 64 - DNA, 336 bp, synthetic construct
  misc_feature 1..336: note = Description of Artificial Sequence: Synthetic polynucleotide
  source 1..336: mol_type = other DNA
caggctgtgctgactcagccaccctcagcgtctgggacccccgggcagagggtcaccatctcttgttctggaagcagctccaacatcggaagtaattacgtattctggtaccagcagctcccaggaacggcccccaaactcctcatctatagtaataatcagcggccctcaggggtccctgaccgattctctggctccaagtctggcacctcagcctccctggccatcagtgggctccggtccgaggatgaggctgattattactgtgcagcatgggatgacagcctgagtgcctcttatgttttcggaactgggaccaaggtcaccgtcctaggt

SEQ ID NO: 65 - protein, 116 aa, synthetic construct
  REGION 1..116: note = Description of Artificial Sequence: Synthetic polypeptide
EVQLVQSGAEVKKPGESLKISCKGSGYSFTSYWIGWVRQMPGKGLEWMGIIYPGDSDTRYSPSFQGHVTISADKSISTAYLQWSSLKASDTAMYYCARYSGSFDNWGQGTLVTVSS

SEQ ID NO: 66 - protein, 111 aa, synthetic construct
  REGION 1..111: note = Description of Artificial Sequence: Synthetic polypeptide
SYELTQPPSASGTPGQRVTMSCSGTSSNIGSHSVNWYQQLPGTAPKLLIYTNNQRPSGVPDRFSGSKSGTSASLAISGLQSEDEADYYCAAWDGSLNGLVFGGGTKLTVLG

SEQ ID NO: 67 - DNA, 348 bp, synthetic construct
  misc_feature 1..348: note = Description of Artificial Sequence: Synthetic polynucleotide
  source 1..348: mol_type = other DNA
gaggtgcagctggtgcagtctggagcagaggtgaaaaagcccggggagtctctgaagatctcctgtaagggttctggatacagctttaccagctactggatcggctgggtgcgccagatgcccgggaaaggcctggagtggatggggatcatctatcctggtgactctgataccagatacagcccgtccttccaaggccacgtcaccatctcagctgacaagtccatcagcactgcctacctgcagtggagcagcctgaaggcctcggacaccgccatgtattactgtgcgcgctactctggttctttcgataactggggtcaaggtactctggtgaccgtctcctca

SEQ ID NO: 68 - DNA, 333 bp, synthetic construct
  misc_feature 1..333: note = Description of Artificial Sequence: Synthetic polynucleotide
  source 1..333: mol_type = other DNA
tcctatgagctgactcagccaccctcagcgtctgggacccccgggcagagggtcaccatgtcttgttctggaaccagctccaacatcggaagtcactctgtaaactggtaccagcagctcccaggaacggcccccaaactcctcatctatactaataatcagcggccctcaggggtccctgaccgattctctggctccaagtctggcacctcagcctccctggccatcagtggcctccagtctgaggatgaggctgattattactgtgcagcatgggatggcagcctgaatggtctggtattcggcggagggaccaagctgaccgtcctaggt

SEQ ID NO: 69 - protein, 21 aa, synthetic construct
  REGION 1..21: note = Description of Artificial Sequence: Synthetic peptide
SRGGGGSGGGGSGGGGSLEMA

SEQ ID NO: 70 - DNA, 63 bp, synthetic construct
  misc_feature 1..63: note = Description of Artificial Sequence: Synthetic oligonucleotide
  source 1..63: mol_type = other DNA
tctagaggtggtggtggtagcggcggcggcggctctggtggtggtggatccctcgagatggcc

SEQ ID NO: 71 - protein, 184 aa, Homo sapiens
MLQMAGQCSQNEYFDSLLHACIPCQLRCSSNTPPLTCQRYCNASVTNSVKGTNAILWTCLGLSLIISLAVFVLMFLLRKINSEPLKDEFKNTGSGLLGMANIDLEKSRTGDEIILPRGLEYTVEECTCEDCIKSKPKVDSDHCFPLPAMEEGATILVTTKTNDYCKSLPAALSATEIEKSISAR

SEQ ID NO: 72 - protein, 255 aa, synthetic construct
  REGION 1..255: note = Description of Artificial Sequence: Synthetic polypeptide
QSVLTQPPSVSVAPRQRVTISCSGSSSNIGHNDVSWYQHLPGKAPRLLIYFDDLLPSGVSDRFSASKSGTSASLAISGLQSEDEADYYCAAWDGSLNAFVFGTGTKVTVLGSRGGGGSGGGGSGGGGSLEMAQVQLQQSGPGLVKPSQTLSLTCAISGDSVSSNSAAWNWIRQSPSRGLEWLGRTYYRSKWYNDYAVSVKSRITINPDTSKNQFSLQLNSVTPEDTAVYYCARQGYSYYGYSDVWGQGTLVTVSS

SEQ ID NO: 73 - protein, 255 aa, synthetic construct
  REGION 1..255: note = Description of Artificial Sequence: Synthetic polypeptide
QPVLTQPPSVSEAPRQRVTISCSGSSSNIGNNAVNWYQQLPGKAPKLLIYFDDLLSSGVSDRFSGSKSGTSASLAISGLQSEDEADYYCAAWDDSLNGYVFGTGTKVTVLGSRGGGGSGGGGSGGGGSLEMAQVQLQQSGPGLVKPSQTLSLTCAISGDSVSSNSAAWNWIRQSPSRGLEWLGRTYYRSKWYNDYAVSVKSRITINPDTSKNQFSLQLNSVTPEDTAVYYCARYGFSGSRFYDTWGQGTLVTVSS

SEQ ID NO: 74 - protein, 254 aa, synthetic construct
  REGION 1..254: note = Description of Artificial Sequence: Synthetic polypeptide
LPVLTQPPSTSGTPGQRVTVSCSGSSSNIGSNVVFWYQQLPGTAPKLVIYRNNQRPSGVPDRFSVSKSGTSASLAISGLRSEDEADYYCAAWDDSLSGYVFGTGTKVTVLGSRGGGGSGGGGSGGGGSLEMAEVQLVQSGAEVKKPGSSVKVSCKASGGTFSSYAISWVRQAPGQGLEWMGRIIPILGIANYAQKFQGRVTMTEDTSTDTAYMELSSLRSEDTAVYYCARSGYSKSIVSYMDYWGQGTLVTVSS

SEQ ID NO: 75 - protein, 251 aa, synthetic construct
  REGION 1..251: note = Description of Artificial Sequence: Synthetic polypeptide
QSVVTQPPSVSGAPGQRVTISCSGSSSNIGARYDVQWYQQLPGTAPKLLIFGNNNRPSGVPDRFSGSKSGTSASLAITGLQAEDEADYYCQSYDSSLSASVFGGGTKLTVLGSRGGGGSGGGGSGGGGSLEMAEVQLVQSGAEVKKPGASVKVSCKASGYTFTSYYMHWVRQAPGQGLEWMGIINPSGGSTSYAQKFQGRVTMTRDTSTSTVYMELSSLRSEDTAVYYCARSQWGGVLDYWGQGTLVTVSS

SEQ ID NO: 76 - protein, 255 aa, synthetic construct
  REGION 1..255: note = Description of Artificial Sequence: Synthetic polypeptide
QAVLTQPPSASGTPGQRVTISCSGSSSNIGSNTVNWYRQLPGTAPKLLIYSNNQRPSGVPDRFSGSKSGTSASLAISGLQSEDEADYYCAAWDDSLNGVVFGGGTKLTVLGSRGGGGSGGGGSGGGGSLEMAQVQLVESGAEVKKPGSSVKVSCKASGGTFSSYAISWVRQAPGQGLEWMGRIIPILGIANYAQKFQGRVTITADESTSTAYMELSSLRSEDTAVYYCARTGYESWGSYEVIDRWGQGTLVTVSS

SEQ ID NO: 77 - protein, 254 aa, synthetic construct
  REGION 1..254: note = Description of Artificial Sequence: Synthetic polypeptide
LPVLTQPPSASGTPGQRVTISCSGRSSNIGSNSVNWYRQLPGAAPKLLIYSNNQRPPGVPVRFSGSKSGTSASLAISGLQSEDEATYYCATWDDNLNVHYVFGTGTKVTVLGSRGGGGSGGGGSGGGGSLEMAQVQLVQSGAEVKKPGSSVKVSCKASGGTFSSYAISWVRQAPGQGLEWMGRIIPILGIANYAQKFQGRVTITADKSTSTAYMELSSLRSEDTAVYYCARGGYYSHDMWSEDWGQGTLVTVSS

SEQ ID NO: 78 - protein, 263 aa, synthetic construct
  REGION 1..263: note = Description of Artificial Sequence: Synthetic polypeptide
QPVLTQPPSASASLGASVTLTCTLSSGYSNYKVDWYQQRPGKGPRFVMRVGTGGIVGSKGDGIPDRFSVLGSGLNRYLTIKNIQEEDEGDYHCGADHGSGSNFVYVFGTGTKVTVLGSRGGGGSGGGGSGGGGSLEMAQVQLQESGPGLVKPSGTLSLTCGVSGGSISNSNWWSWVRQPPGKGLEWIGEIYHSGSTKYNPSLRSRVTISVDKSKNQFSLKLSSVTAADTAVYYCARRDNWKTPTTKIDGFDIWGQGTMVTVSS

SEQ ID NO: 79 - protein, 247 aa, synthetic construct
  REGION 1..247: note = Description of Artificial Sequence: Synthetic polypeptide
DIQLTQSPSSLSASVGDRVTITCRASQSISSYLNWYQQKPGKAPKLLIYAASSLQSGVPSRFSGSGSGTDFTLTISSLQPEDFATYYCQQSYSTPPTFGQGTKVEIKRSRGGGGSGGGGSGGGGSLEMAQVQLVQSGAEVKKPGASVKVSCKASGYTFTGYYMHWVRQAPGQGLEWMGWINPNSGGTNYAQKFQGRVTMTRDTSISTAYMELSRLRSDDTAVYYCARSQWGSSWDYWGQGTLVTVSS

SEQ ID NO: 80 - protein, 257 aa, synthetic construct
  REGION 1..257: note = Description of Artificial Sequence: Synthetic polypeptide
QPVLTQPPSASASLGASVTLTCTLSNDYTNYKVDWYQQRPGKGPRFVMRVGPGGIVGSKGDGIPDRFSVLGSGLNRYLTIKNIQEEDESDYHCGADHGTGSNFVYVFGGGTKLTVLGSRGGGGSGGGGSGGGGSLEMAEVQLVESGAEVKKPGASVKVSCKASGYTFTGYYMHWVRQAPGQGLEWMGWINPNSGGTNYAQKFQGRVTMTRDTSISTAYMELSRLRSDDTAVYYCARSSYHLYGYDSWGQGTLVTVSS

SEQ ID NO: 81 - protein, 258 aa, synthetic construct
  REGION 1..258: note = Description of Artificial Sequence: Synthetic polypeptide
QPVLTQPPSASASLGASVTLTCTLSSGYSNYKVDWYQQRPGKGPRFLMRVDTGGIVGSKGDGIPDRFSVSGSGLNRYLTIKNIQEEDESDYHCGADHGSGSNFVWVFGGGTKLTVLGSRGGGGSGGGGSGGGGSLEMAQVQLVQSGAEVKKPGSSVKVSCKASGGTFSSYAISWVRQAPGQGLEWMGGIIPIFSTANYAQKFQGRVTMTTDTSTSTAYMELRSLRSDDTAVYYCARQPWTWYSPYDQWGQGTLVTVSS

SEQ ID NO: 82 - protein, 251 aa, synthetic construct
  REGION 1..251: note = Description of Artificial Sequence: Synthetic polypeptide
DVVMTQSPLSLPVTPGEPASISCRSSQSLLHSNGYNYLDWYLQKPGQSPQLLIYLGSNRASGVPDRFSGSGSGTDFTLKISRVEAEDVGVYYCMQALQTPLTFGGGTKVEIKRSRGGGGSGGGGSGGGGSLEMAEVQLVETGGGLVQPGGSLRLSCAASGFTFSTYAMTWVRQAPGKGLEWVSAITPGGDRTYYADSVKGRFTISRDNSRNTLYLQMNSLRAEDTAVYYCARYYGYMIDMWGQGTLVTVSS

SEQ ID NO: 83 - protein, 250 aa, synthetic construct
  REGION 1..250: note = Description of Artificial Sequence: Synthetic polypeptide
SYVLTQPPSASGTPGQRVTISCSGSSSNIGSNTVNWYQQVPGTAPKLLIYSNNQRPSGVPDRFSGSKSGASASLAISWLQSEDEADYYCAAWDDSLNGWVFGGGTKLTVLGSRGGGGSGGGGSGGGGSLEMAQMQLVQSGAEVKKPGASVKVSCKASGYTFTGYYVHWLRQAPGQGLEWMGWINPNSGGTNNAQEFQGRITMTRDTSINTAYMELSRLRSDDTAVYYCARSQWGGTYDYWGQGTLVTVSS

SEQ ID NO: 84 - protein, 249 aa, synthetic construct
  REGION 1..249: note = Description of Artificial Sequence: Synthetic polypeptide
QAVLTQPPSASGTPGQRVTISCSGSSSNIGSYTVSWYQQLPGTAPKFLIYSNNQRPSGVPDRFSGSKSGTSASLAISGLQSEDEADYYCAAWDDSLNGYVFGTGTKVTVLGSRGGGGSGGGGSGGGGSLEMAEVQLVQSGAEVKKPGESLKISCKGSGYDFTTYWIGWVRQMPGKGLEWMGIIYPGDSDTRYSPSVRGRVTISADKSINTAYLQWSSLEASDTAMYYCARMWTFSQDGWGQGTLVTVSS

SEQ ID NO: 85 - protein, 244 aa, synthetic construct
  REGION 1..244: note = Description of Artificial Sequence: Synthetic polypeptide
QSALTQPASVSASPGQSIAISCTGTSSDVGWYQQHPGKAPKLMIYEDSKRPSGVSNRFSGSKSGNTASLTISGLQAEDEADYYCSSNTRSSTLVFGGGTKLTVLGSRGGGGSGGGGSGGGGSLEMAEVQLVQSGAEMKKPGASLKLSCKASGYTFIDYYVYWMRQAPGQGLESMGWINPNSGGTNYAQKFQGRVTMTRDTSISTAYMELSRLRSDDTAMYYCARSQRDGYMDYWGQGTLVTVSS

SEQ ID NO: 86 - protein, 251 aa, synthetic construct
  REGION 1..251: note = Description of Artificial Sequence: Synthetic polypeptide
QSVLTQPPSVSGAPGQRVTISCTGSSSNIGAGFDVHWYQQLPGTAPKLLIYGNSNRPSGVPDRFSGSKSGTSASLAITGLQAEDEADYYCQSYDSSLSGYVFGTGTKVTVLGSRGGGGSGGGGSGGGGSLEMAQVQLVQSGAEVKKPGASVKVSCKASGYTFTDYYMHWVRQAPGQRLEWMGWINPNSGGTNYAQKFQDRITVTRDTSSNTGYMELTRLRSDDTAVYYCARSPYSGVLDKWGQGTLVTVSS

SEQ ID NO: 87 - protein, 253 aa, synthetic construct
  REGION 1..253: note = Description of Artificial Sequence: Synthetic polypeptide
QAVLTQPPSASGTPGQRVTISCSGSSSNIGSNYVFWYQQLPGTAPKLLIYSNNQRPSGVPDRFSGSKSGTSASLAISGLRSEDEADYYCAAWDDSLSASYVFGTGTKVTVLGSRGGGGSGGGGSGGGGSLEMAQVQLVQSGAEVKKPGSSVKVSCKASGGTFSSYAISWVRQAPGQGLEWMGRIIPILGTANYAQKFQGRVTITADESTSTAYMELSSLRSEDTAVYYCARSGYGSYRWEDSWGQGTLVTVSS

SEQ ID NO: 88 - protein, 248 aa, synthetic construct
  REGION 1..248: note = Description of Artificial Sequence: Synthetic polypeptide
SYELTQPPSASGTPGQRVTMSCSGTSSNIGSHSVNWYQQLPGTAPKLLIYTNNQRPSGVPDRFSGSKSGTSASLAISGLQSEDEADYYCAAWDGSLNGLVFGGGTKLTVLGSRGGGGSGGGGSGGGGSLEMAEVQLVQSGAEVKKPGESLKISCKGSGYSFTSYWIGWVRQMPGKGLEWMGIIYPGDSDTRYSPSFQGHVTISADKSISTAYLQWSSLKASDTAMYYCARYSGSFDNWGQGTLVTVSS

SEQ ID NO: 89 - protein, 9 aa, synthetic construct
  REGION 1..9: note = Description of Artificial Sequence: Synthetic peptide
VSSNSAAWN

SEQ ID NO: 90 - protein, 7 aa, synthetic construct
  REGION 1..7: note = Description of Artificial Sequence: Synthetic peptide
YRSKWYN

SEQ ID NO: 91 - protein, 13 aa, synthetic construct
  REGION 1..13: note = Description of Artificial Sequence: Synthetic peptide
ARQGYSYYGYSDV

SEQ ID NO: 92 - protein, 8 aa, synthetic construct
  REGION 1..8: note = Description of Artificial Sequence: Synthetic peptide
SSNIGHND

SEQ ID NO: 93 - skipped

SEQ ID NO: 94 - protein, 11 aa, synthetic construct
  REGION 1..11: note = Description of Artificial Sequence: Synthetic peptide
AAWDGSLNAFV

SEQ ID NO: 95 - protein, 9 aa, synthetic construct
  REGION 1..9: note = Description of Artificial Sequence: Synthetic peptide
VSSNSAAWN

SEQ ID NO: 96 - protein, 7 aa, synthetic construct
  REGION 1..7: note = Description of Artificial Sequence: Synthetic peptide
YRSKWYN

SEQ ID NO: 97 - protein, 13 aa, synthetic construct
  REGION 1..13: note = Description of Artificial Sequence: Synthetic peptide
ARYGFSGSRFYDT

SEQ ID NO: 98 - protein, 8 aa, synthetic construct
  REGION 1..8: note = Description of Artificial Sequence: Synthetic peptide
SSNIGNNA

SEQ ID NO: 99 - skipped

SEQ ID NO: 100 - protein, 11 aa, synthetic construct
  REGION 1..11: note = Description of Artificial Sequence: Synthetic peptide
AAWDDSLNGYV

SEQ ID NO: 101 - protein, 8 aa, synthetic construct
  REGION 1..8: note = Description of Artificial Sequence: Synthetic peptide
GGTFSSYA

SEQ ID NO: 102 - protein, 8 aa, synthetic construct
  REGION 1..8: note = Description of Artificial Sequence: Synthetic peptide
IIPILGIA

SEQ ID NO: 103 - protein, 15 aa, synthetic construct
  REGION 1..15: note = Description of Artificial Sequence: Synthetic peptide
ARSGYSKSIVSYMDY

SEQ ID NO: 104 - protein, 8 aa, synthetic construct
  REGION 1..8: note = Description of Artificial Sequence: Synthetic peptide
SSNIGSNV

SEQ ID NO: 105 - skipped

SEQ ID NO: 106 - protein, 11 aa, synthetic construct
  REGION 1..11: note = Description of Artificial Sequence: Synthetic peptide
AAWDDSLSGYV

SEQ ID NO: 107 - protein, 8 aa, synthetic construct
  REGION 1..8: note = Description of Artificial Sequence: Synthetic peptide
GYTFTSYY

SEQ ID NO: 108 - protein, 8 aa, synthetic construct
  REGION 1..8: note = Description of Artificial Sequence: Synthetic peptide
INPSGGST

SEQ ID NO: 109 - protein, 11 aa, synthetic construct
  REGION 1..11: note = Description of Artificial Sequence: Synthetic peptide
ARSQWGGVLDY

SEQ ID NO: 110 - protein, 9 aa, synthetic construct
  REGION 1..9: note = Description of Artificial Sequence: Synthetic peptide
SSNIGARYD

SEQ ID NO: 111 - skipped

SEQ ID NO: 112 - protein, 11 aa, synthetic construct
  REGION 1..11: note = Description of Artificial Sequence: Synthetic peptide
QSYDSSLSASV

SEQ ID NO: 113 - protein, 8 aa, synthetic construct
  REGION 1..8: note = Description of Artificial Sequence: Synthetic peptide
GGTFSSYA

SEQ ID NO: 114 - protein, 8 aa, synthetic construct
  REGION 1..8: note = Description of Artificial Sequence: Synthetic peptide
IIPILGIA

SEQ ID NO: 115 - protein, 16 aa, synthetic construct
  REGION 1..16: note = Description of Artificial Sequence: Synthetic peptide
ARTGYESWGSYEVIDR

SEQ ID NO: 116 - protein, 8 aa, synthetic construct
  REGION 1..8: note = Description of Artificial Sequence: Synthetic peptide
SSNIGSNT

SEQ ID NO: 117 - skipped

SEQ ID NO: 118 - protein, 11 aa, synthetic construct
  REGION 1..11: note = Description of Artificial Sequence: Synthetic peptide
AAWDDSLNGVV

SEQ ID NO: 119 - protein, 8 aa, synthetic construct
  REGION 1..8: note = Description of Artificial Sequence: Synthetic peptide
GGTFSSYA

SEQ ID NO: 120 - protein, 8 aa, synthetic construct
  REGION 1..8: note = Description of Artificial Sequence: Synthetic peptide
IIPILGIA

SEQ ID NO: 121 - protein, 14 aa, synthetic construct
  REGION 1..14: note = Description of Artificial Sequence: Synthetic peptide
ARGGYYSHDMWSED

SEQ ID NO: 122 - protein, 8 aa, synthetic construct
  REGION 1..8: note = Description of Artificial Sequence: Synthetic peptide
SSNIGSNS

SEQ ID NO: 123 - skipped

SEQ ID NO: 124 - protein, 12 aa, synthetic construct
  REGION 1..12: note = Description of Artificial Sequence: Synthetic peptide
ATWDDNLNVHYV

SEQ ID NO: 125 - protein, 9 aa, synthetic construct
  REGION 1..9: note = Description of Artificial Sequence: Synthetic peptide
GGSISNSNW

SEQ ID NO: 126 - protein, 7 aa, synthetic construct
  REGION 1..7: note = Description of Artificial Sequence: Synthetic peptide
IYHSGST

SEQ ID NO: 127 - protein, 18 aa, synthetic construct
  REGION 1..18: note = Description of Artificial Sequence: Synthetic peptide
ARRDNWKTPTTKIDGFDI

SEQ ID NO: 128 - protein, 7 aa, synthetic construct
  REGION 1..7: note = Description of Artificial Sequence: Synthetic peptide
SGYSNYK

SEQ ID NO: 129 - protein, 8 aa, synthetic construct
  REGION 1..8: note = Description of Artificial Sequence: Synthetic peptide
VGTGGIVG

SEQ ID NO: 130 - protein, 13 aa, synthetic construct
  REGION 1..13: note = Description of Artificial Sequence: Synthetic peptide
GADHGSGSNFVYV

SEQ ID NO: 131 - protein, 8 aa, synthetic construct
  REGION 1..8: note = Description of Artificial Sequence: Synthetic peptide
GYTFTGYY

SEQ ID NO: 132 - protein, 8 aa, synthetic construct
  REGION 1..8: note = Description of Artificial Sequence: Synthetic peptide
INPNSGGT

SEQ ID NO: 133 - protein, 11 aa, synthetic construct
  REGION 1..11: note = Description of Artificial Sequence: Synthetic peptide
ARSQWGSSWDY

SEQ ID NO: 134 - protein, 6 aa, synthetic construct
  REGION 1..6: note = Description of Artificial Sequence: Synthetic peptide
QSISSY

SEQ ID NO: 135 - skipped

SEQ ID NO: 136 - protein, 9 aa, synthetic construct
  REGION 1..9: note = Description of Artificial Sequence: Synthetic peptide
QQSYSTPPT

SEQ ID NO: 137 - protein, 8 aa, synthetic construct
  REGION 1..8: note = Description of Artificial Sequence: Synthetic peptide
GYTFTGYY

SEQ ID NO: 138 - protein, 8 aa, synthetic construct
  REGION 1..8: note = Description of Artificial Sequence: Synthetic peptide
INPNSGGT

SEQ ID NO: 139 - protein, 12 aa, synthetic construct
  REGION 1..12: note = Description of Artificial Sequence: Synthetic peptide
ARSSYHLYGYDS

SEQ ID NO: 140 - protein, 7 aa, synthetic construct
  REGION 1..7: note = Description of Artificial Sequence: Synthetic peptide
NDYTNYK

SEQ ID NO: 141 - protein, 8 aa, synthetic construct
  REGION 1..8: note = Description of Artificial Sequence: Synthetic peptide
VGPGGIVG

SEQ ID NO: 142 - protein, 13 aa, synthetic construct
  REGION 1..13: note = Description of Artificial Sequence: Synthetic peptide
GADHGTGSNFVYV

SEQ ID NO: 143 - protein, 8 aa, synthetic construct
  REGION 1..8: note = Description of Artificial Sequence: Synthetic peptide
GGTFSSYA

SEQ ID NO: 144 - protein, 8 aa, synthetic construct
  REGION 1..8: note = Description of Artificial Sequence: Synthetic peptide
IIPIFSTA

SEQ ID NO: 145 - protein, 13 aa, synthetic construct
  REGION 1..13: note = Description of Artificial Sequence: Synthetic peptide
ARQPWTWYSPYDQ

SEQ ID NO: 146 - protein, 7 aa, synthetic construct
  REGION 1..7: note = Description of Artificial Sequence: Synthetic peptide
SGYSNYK

SEQ ID NO: 147 - protein, 8 aa, synthetic construct
  REGION 1..8: note = Description of Artificial Sequence: Synthetic peptide
VDTGGIVG

SEQ ID NO: 148 - protein, 13 aa, synthetic construct
  REGION 1..13: note = Description of Artificial Sequence: Synthetic peptide
GADHGSGSNFVWV

SEQ ID NO: 149 - protein, 8 aa, synthetic construct
  REGION 1..8: note = Description of Artificial Sequence: Synthetic peptide
GFTFSTYA

SEQ ID NO: 150 - protein, 8 aa, synthetic construct
  REGION 1..8: note = Description of Artificial Sequence: Synthetic peptide
ITPGGDRT

SEQ ID NO: 151 - protein, 10 aa, synthetic construct
  REGION 1..10: note = Description of Artificial Sequence: Synthetic peptide
ARYYGYMIDM

SEQ ID NO: 152 - protein, 11 aa, synthetic construct
  REGION 1..11: note = Description of Artificial Sequence: Synthetic peptide
QSLLHSNGYNY

SEQ ID NO: 153 - skipped

SEQ ID NO: 154 - protein, 9 aa, synthetic construct
  REGION 1..9: note = Description of Artificial Sequence: Synthetic peptide
MQALQTPLT

SEQ ID NO: 155 - protein, 8 aa, synthetic construct
  REGION 1..8: note = Description of Artificial Sequence: Synthetic peptide
GYTFTGYY

SEQ ID NO: 156 - protein, 8 aa, synthetic construct
  REGION 1..8: note = Description of Artificial Sequence: Synthetic peptide
INPNSGGT

SEQ ID NO: 157 - protein, 11 aa, synthetic construct
  REGION 1..11: note = Description of Artificial Sequence: Synthetic peptide
ARSQWGGTYDY

SEQ ID NO: 158 - protein, 8 aa, synthetic construct
  REGION 1..8: note = Description of Artificial Sequence: Synthetic peptide
SSNIGSNT

SEQ ID NO: 159 - skipped

SEQ ID NO: 160 - protein, 11 aa, synthetic construct
  REGION 1..11: note = Description of Artificial Sequence: Synthetic peptide
AAWDDSLNGWV

SEQ ID NO: 161 - protein, 8 aa, synthetic construct
  REGION 1..8: note = Description of Artificial Sequence: Synthetic peptide
GYDFTTYW

SEQ ID NO: 162 - protein, 8 aa, synthetic construct
  REGION 1..8: note = Description of Artificial Sequence: Synthetic peptide
IYPGDSDT

SEQ ID NO: 163 - protein, 10 aa, synthetic construct
  REGION 1..10: note = Description of Artificial Sequence: Synthetic peptide
ARMWTFSQDG

SEQ ID NO: 164 - protein, 8 aa, synthetic construct
  REGION 1..8: note = Description of Artificial Sequence: Synthetic peptide
SSNIGSYT

SEQ ID NO: 165 - skipped

SEQ ID NO: 166 - protein, 11 aa, synthetic construct
  REGION 1..11: note = Description of Artificial Sequence: Synthetic peptide
AAWDDSLNGYV

SEQ ID NO: 167 - protein, 8 aa, synthetic construct
  REGION 1..8: note = Description of Artificial Sequence: Synthetic peptide
GYTFIDYY

SEQ ID NO: 168 - protein, 8 aa, synthetic construct
  REGION 1..8: note = Description of Artificial Sequence: Synthetic peptide
INPNSGGT

SEQ ID NO: 169 - protein, 11 aa, synthetic construct
  REGION 1..11: note = Description of Artificial Sequence: Synthetic peptide
ARSQRDGYMDY

SEQ ID NO: 170 - protein, 9 aa, synthetic construct
  REGION 1..9: note = Description of Artificial Sequence: Synthetic peptide
ISCTGTSSD

SEQ ID NO: 171 - skipped

SEQ ID NO: 172 - protein, 10 aa, synthetic construct
  REGION 1..10: note = Description of Artificial Sequence: Synthetic peptide
SSNTRSSTLV

SEQ ID NO: 173 - protein, 8 aa, synthetic construct
  REGION 1..8: note = Description of Artificial Sequence: Synthetic peptide
GYTFTDYY

SEQ ID NO: 174 - protein, 8 aa, synthetic construct
  REGION 1..8: note = Description of Artificial Sequence: Synthetic peptide
INPNSGGT

SEQ ID NO: 175 - protein, 11 aa, synthetic construct
  REGION 1..11: note = Description of Artificial Sequence: Synthetic peptide
ARSPYSGVLDK

SEQ ID NO: 176 - protein, 9 aa, synthetic construct
  REGION 1..9: note = Description of Artificial Sequence: Synthetic peptide
SSNIGAGFD

SEQ ID NO: 177 - skipped

SEQ ID NO: 178 - protein, 11 aa, synthetic construct
  REGION 1..11: note = Description of Artificial Sequence: Synthetic peptide
QSYDSSLSGYV

SEQ ID NO: 179 - protein, 8 aa, synthetic construct
  REGION 1..8: note = Description of Artificial Sequence: Synthetic peptide
GGTFSSYA

SEQ ID NO: 180 - protein, 8 aa, synthetic construct
  REGION 1..8: note = Description of Artificial Sequence: Synthetic peptide
IIPILGTA

SEQ ID NO: 181 - protein, 13 aa, synthetic construct
  REGION 1..13: note = Description of Artificial Sequence: Synthetic peptide
ARSGYGSYRWEDS

SEQ ID NO: 182 - protein, 8 aa, synthetic construct
  REGION 1..8: note = Description of Artificial Sequence: Synthetic peptide
SSNIGSNY

SEQ ID NO: 183 - skipped

SEQ ID NO: 184 - protein, 12 aa, synthetic construct
  REGION 1..12: note = Description of Artificial Sequence: Synthetic peptide
AAWDDSLSASYV

SEQ ID NO: 185 - protein, 8 aa, synthetic construct
  REGION 1..8: note = Description of Artificial Sequence: Synthetic peptide
GYSFTSYW

SEQ ID NO: 186 - protein, 8 aa, synthetic construct
  REGION 1..8: note = Description of Artificial Sequence: Synthetic peptide
IYPGDSDT

SEQ ID NO: 187 - protein, 9 aa, synthetic construct
  REGION 1..9: note = Description of Artificial Sequence: Synthetic peptide
ARYSGSFDN

SEQ ID NO: 188 - protein, 8 aa, synthetic construct
  REGION 1..8: note = Description of Artificial Sequence: Synthetic peptide
SSNIGSHS

SEQ ID NO: 189 - skipped

SEQ ID NO: 190 - protein, 11 aa, synthetic construct
  REGION 1..11: note = Description of Artificial Sequence: Synthetic peptide
AAWDGSLNGLV

SEQ ID NO: 191 - protein, 20 aa, synthetic construct
  REGION 1..20: note = Description of Artificial Sequence: Synthetic peptide
MALPVTALLLPLALLLHAAR

SEQ ID NO: 192 - DNA, 60 bp, synthetic construct
  misc_feature 1..60: note = Description of Artificial Sequence: Synthetic oligonucleotide
  source 1..60: mol_type = other DNA
atggctctcccagtgactgccctactgcttcccctagcgcttctcctgcatgcagctcgt

SEQ ID NO: 193 - protein, 220 aa, Homo sapiens
MLRLLLALNLFPSIQVTGNKILVKQSPMLVAYDNAVNLSCKYSYNLFSREFRASLHKGLDSAVEVCVVYGNYSQQLQVYSKTGFNCDGKLGNESVTFYLQNLYVNQTDIYFCKIEVMYPPPYLDNEKSNGTIIHVKGKHLCPSPLFPGPSKPFWVLVVVGGVLACYSLLVTVAFIIFWVRSKRSRLLHSDYMNMTPRRPGPTRKHYQPYAPPRDFAAYRS

SEQ ID NO: 194 - DNA, 321 bp, Homo sapiens
  source 1..321: mol_type = other DNA
attgaagttatgtatcctcctccttacctagacaatgagaagagcaatggaaccattatccatgtgaaagggaaacacctttgtccaagtcccctatttcccggaccttctaagcccttttgggtgctggtggtggttggtggagtcctggcttgctatagcttgctagtaacagtggcctttattattttctgggtgaggagtaagaggagcaggctcctgcacagtgactacatgaacatgactccccgccgccccgggcccacccgcaagcattaccagccctatgccccaccacgcgacttcgcagcctatcgctcc

SEQ ID NO: 195 - protein, 163 aa, Homo sapiens
MKWKALFTAAILQAQLPITEAQSFGLLDPKLCYLLDGILFIYGVILTALFLRVKFSRSADAPAYQQGQNQLYNELNLGRREEYDVLDKRRGRDPEMGGKPRRKNPQEGLYNELQKDKMAEAYSEIGMKGERRRGKGHDGLYQGLSTATKDTYDALHMQALPPR

SEQ ID NO: 196 - DNA, 339 bp, Homo sapiens
  source 1..339: mol_type = other DNA
agagtgaagttcagcaggagcgcagacgcccccgcgtaccagcagggccagaaccagctctataacgagctcaatctaggacgaagagaggagtacgatgttttggacaagagacgtggccgggaccctgagatggggggaaagccgagaaggaagaaccctcaggaaggcctgtacaatgaactgcagaaagataagatggcggaggcctacagtgagattgggatgaaaggcgagcgccggaggggcaaggggcacgatggcctttaccagggtctcagtacagccaccaaggacacctacgacgcccttcacatgcaggccctgccccctcgctaa

SEQ ID NO: 197 - protein, 255 aa, Homo sapiens
MGNSCYNIVATLLLVLNFERTRSLQDPCSNCPAGTFCDNNRNQICSPCPPNSFSSAGGQRTCDICRQCKGVFRTRKECSSTSNAECDCTPGFHCLGAGCSMCEQDCKQGQELTKKGCKDCCFGTFNDQKRGICRPWTNCSLDGKSVLVNGTKERDVVCGPSPADLSPGASSVTPPAPAREPGHSPQIISFFLALTSTALLFLLFFLTLRFSVVKRGRKKLLYIFKQPFMRPVQTTQEEDGCSCRFPEEEEGGCEL

SEQ ID NO: 198 - protein, 277 aa, Homo sapiens
MCVGARRLGRGPCAALLLLGLGLSTVTGLHCVGDTYPSNDRCCHECRPGNGMVSRCSRSQNTVCRPCGPGFYNDVVSSKPCKPCTWCNLRSGSERKQLCTATQDTVCRCRAGTQPLDSYKPGVDCAPCPPGHFSPGDNQACKPWTNCTLAGKHTLQPASNSSDAICEDRDPPATQPQETQGPPARPITVQPTEAWPRTSQGPSTRPVEVPGGRAVAAILGLGLVLGLLGPLAILLALYLLRRDQRLPPDAHKPPGGGSFRTPIQEEQADAHSTLAKI

SEQ ID NO: 199 - protein, 199 aa, Homo sapiens
MKSGLWYFFLFCLRIKVLTGEINGSANYEMFIFHNGGVQILCKYPDIVQQFKMQLLKGGQILCDLTKTKGSGNTVSIKSLKFCHSQLSNNSVSFFLYNLDHSHANYYFCNLSIFDPPPFKVTLTGGYLHIYESQLCCQLKFWLPIGCAAFVVVCILGCILICWLTKKKYSSSVHDPNGEYMFMRAVNTAKKSRLTDVTL

SEQ ID NO: 200 - protein, 223 aa, Homo sapiens
MACLGFQRHKAQLNLATRTWPCTLLFFLLFIPVFCKAMHVAQPAVVLASSRGIASFVCEYASPGKATEVRVTVLRQADSQVTEVCAATYMMGNELTFLDDSICTGTSSGNQVNLTIQGLRAMDTGLYICKVELMYPPPYYLGIGNGTQIYVIDPEPCPDSDFLLWILAAVSSGLFFYSFLLTAVSLSKMLKKRSPLTTGVYVKMPPTEPECEKQFQPYFIPIN

SEQ ID NO: 201 - protein, 288 aa, Homo sapiens
MQIPQAPWPVVWAVLQLGWRPGWFLDSPDRPWNPPTFSPALLVVTEGDNATFTCSFSNTSESFVLNWYRMSPSNQTDKLAAFPEDRSQPGQDCRFRVTQLPNGRDFHMSVVRARRNDSGTYLCGAISLAPKAQIKESLRAELRVTERRAEVPTAHPSPSPRPAGQFQTLVVGVVGGLLGSLVLLVWVLAVICSRAARGTIGARRTGQPLKEDPSAVPVFSVDYGELDFQWREKTPEPPVPCVPEQTEYATIVFPSGMGTSSPARRGSADGPRSAQPLRPEDGHCSWPL

SEQ ID NO: 202 - protein, 525 aa, Homo sapiens
MWEAQFLGLLFLQPLWVAPVKPLQPGAEVPVVWAQEGAPAQLPCSPTIPLQDLSLLRRAGVTWQHQPDSGPPAAAPGHPLAPGPHPAAPSSWGPRPRRYTVLSVGPGGLRSGRLPLQPRVQLDERGRQRGDFSLWLRPARRADAGEYRAAVHLRDRALSCRLRLRLGQASMTASPPGSLRASDWVILNCSFSRPDRPASVHWFRNRGQGRVPVRESPHHHLAESFLFLPQVSPMDSGPWGCILTYRDGFNVSIMYNLTVLGLEPPTPLTVYAGAGSRVGLPCRLPAGVGTRSFLTAKWTPPGGGPDLLVTGDNGDFTLRLEDVSQAQAGTYTCHIHLQEQQLNATVTLAIITVTPKSFGSPGSLGKLLCEVTPVSGQERFVWSSLDTPSQRSFSGPWLEAQEAQLLSQPWQCQLYQGERLLGAAVYFTELSSPGAQRSGRAPGALPAGHLLLFLILGVLSLLLLVTGAFGFHLWRRQWRPRRFSALEQGIHPPQAQSKIEELEQEPEPEPEPEPEPEPEPEPEQL

SEQ ID NO: 203 - protein, 370 aa, Homo sapiens
MLGQVVTLILLLLLKVYQGKGCQGSADHVVSISGVPLQLQPNSIQTKVDSIAWKKLLPSQNGFHHILKWENGSLPSNTSNDRFSFIVKNLSLLIKAAQQQDSGLYCLEVTSISGKVQTATFQVFVFESLLPDKVEKPRLQGQGKILDRGRCQVALSCLVSRDGNVSYAWYRGSKLIQTAGNLTYLDEEVDINGTHTYTCNVSNPVSWESHTLNLTQDCQNAHQEFRFWPFLVIIVILSALFLGTLACFCVWRRKRKEKQSETSPKEFLTIYEDVKDLKTRRNHEQEQTFPGGGSTIYSMIQSQSSAPTSQEPAYTLYSLIQPSRKSGSRKRNHSPSFNSTIYEVIGKSQPKAQNPARLSRKELENFDVYS

SEQ ID NO: 204 - protein, 289 aa, Homo sapiens
MKTLPAMLGTGKLFWVFFLIPYLDIWNIHGKESCDVQLYIKRQSEHSILAGDPFELECPVKYCANRPHVTWCKLNGTTCVKLEDRQTSWKEEKNISFFILHFEPVLPNDNGSYRCSANFQSNLIESHSTTLYVTDVKSASERPSKDEMASRPWLLYRLLPLGGLPLLITTCFCLFCCLRRHQGKQNELSDTAGREINLVDAHLKSEQTEASTRQNSQVLLSETGIYDNDPDLCFRMQEGSEVYSNPCLEENKPGIVYASLNHSVIGPNSRLARNVKEAPTEYASICVRS

SEQ ID NO: 205 - protein, 20 aa, synthetic construct
  REGION 1..20: note = Description of Artificial Sequence: Synthetic peptide
METDTLLLWVLLLWVPGSTG

SEQ ID NO: 206 - DNA, 60 bp, synthetic construct
  misc_feature 1..60: note = Description of Artificial Sequence: Synthetic oligonucleotide
  source 1..60: mol_type = other DNA
atggaaaccgacaccctgctgctgtgggtgctgctgctgtgggtgccaggatccacagga

SEQ ID NO: 207 - DNA, 1398 bp, synthetic construct
  misc_feature 1..1398: note = Description of Artificial Sequence: Synthetic polynucleotide
  source 1..1398: mol_type = other DNA
caatctgccctgactcagcctgcctccgtgtctgcgtctcctggacagtcgatcgccatctcctgcactggaaccagcagtgacgttggttggtatcaacagcacccaggcaaagcccccaaactcatgatttatgaggacagtaagcggccctcaggggtttctaatcgcttctctggctccaagtctggcaacacggcctccctgaccatctctgggctccaggctgaggacgaggctgattattactgcagctcaaatacaagaagcagcactttggtgttcggcggagggaccaagctgaccgtcctaggttctagaggtggtggtggtagcggcggcggcggctctggtggtggtggatccctcgagatggccgaagtgcagctggtgcagtctggggctgagatgaagaagcctggggcctcactgaagctctcctgcaaggcttctggatacaccttcatcgactactatgtatactggatgcgacaggcccctggacaagggcttgagtccatgggatggatcaaccctaacagtggtggcacaaactatgcacagaagtttcagggcagggtcaccatgaccagggacacgtccatcagcacagcctacatggagctgagcaggctgagatctgacgacaccgccatgtattactgtgcgcgctcccagcgtgacggttacatggattactggggtcaaggtactctggtgaccgtctcctcagcggccgcaattgaagttatgtatcctcctccttacctagacaatgagaagagcaatggaaccattatccatgtgaaagggaaacacctttgtccaagtcccctatttcccggaccttctaagcccttttgggtgctggtggtggttggtggagtcctggcttgctatagcttgctagtaacagtggcctttattattttctgggtgaggagtaagaggagcaggctcctgcacagtgactacatgaacatgactccccgccgccccgggcccacccgcaagcattaccagccctatgccccaccacgcgacttcgcagcctatcgctccagagtgaagttcagcaggagcgcagacgcccccgcgtaccagcagggccagaaccagctctataacgagctcaatctaggacgaagagaggagtacgatgttttggacaagagacgtggccgggaccctgagatggggggaaagccgagaaggaagaaccctcaggaaggcctgtacaatgaactgcagaaagataagatggcggaggcctacagtgagattgggatgaaaggcgagcgccggaggggcaaggggcacgatggcctttaccagggtctcagtacagccaccaaggacacctacgacgcccttcacatgcaggccctgccccctcgc

SEQ ID NO: 208 - DNA, 1419 bp, synthetic construct
  misc_feature 1..1419: note = Description of Artificial Sequence: Synthetic polynucleotide
  source 1..1419: mol_type = other DNA
cagtctgtgctgacgcagccgccctcagtgtctggggccccagggcagagggtcaccatctcctgcactgggagcagctccaacatcggggcaggttttgatgtacactggtaccagcagcttccaggaacagcccccaaactcctcatctatggtaacagcaatcggccctcaggggtccctgaccgattctctggctccaagtctggcacctcagcctccctggccatcactgggctccaggctgaggatgaggctgattattactgccagtcctatgacagcagcctgagtggttatgtcttcggaactgggaccaaggtcaccgtcctaggttctagaggtggtggtggtagcggcggcggcggctctggtggtggtggatccctcgagatggcccaggtccagctggtacagtctggggctgaggtgaagaagcctggggcctcagtgaaggtctcctgcaaggcttctggatacaccttcaccgactactatatgcactgggtgcgacaggcccctggacaacggcttgagtggatgggatggatcaaccctaacagtggtggcacaaactatgcacagaagtttcaggacaggatcaccgtgaccagggacacctccagcaacacaggctacatggagctgaccaggctgagatctgacgacacggccgtgtattactgtgcgcgctctccgtactctggtgttctggataaatggggtcaaggtactctggtgaccgtctcctcagcggccgcaattgaagttatgtatcctcctccttacctagacaatgagaagagcaatggaaccattatccatgtgaaagggaaacacctttgtccaagtcccctatttcccggaccttctaagcccttttgggtgctggtggtggttggtggagtcctggcttgctatagcttgctagtaacagtggcctttattattttctgggtgaggagtaagaggagcaggctcctgcacagtgactacatgaacatgactccccgccgccccgggcccacccgcaagcattaccagccctatgccccaccacgcgacttcgcagcctatcgctccagagtgaagttcagcaggagcgcagacgcccccgcgtaccagcagggccagaaccagctctataacgagctcaatctaggacgaagagaggagtacgatgttttggacaagagacgtggccgggaccctgagatggggggaaagccgagaaggaagaaccctcaggaaggcctgtacaatgaactgcagaaagataagatggcggaggcctacagtgagattgggatgaaaggcgagcgccggaggggcaaggggcacgatggcctttaccagggtctcagtacagccaccaaggacacctacgacgcccttcacatgcaggccctgccccctcgc

SEQ ID NO: 209 - DNA, 1410 bp, synthetic construct
  misc_feature 1..1410: note = Description of Artificial Sequence: Synthetic polynucleotide
  source 1..1410: mol_type = other DNA
tcctatgagctgactcagccaccctcagcgtctgggacccccgggcagagggtcaccatgtcttgttctggaaccagctccaacatcggaagtcactctgtaaactggtaccagcagctcccaggaacggcccccaaactcctcatctatactaataatcagcggccctcaggggtccctgaccgattctctggctccaagtctggcacctcagcctccctggccatcagtggcctccagtctgaggatgaggctgattattactgtgcagcatgggatggcagcctgaatggtctggtattcggcggagggaccaagctgaccgtcctaggttctagaggtggtggtggtagcggcggcggcggctctggtggtggtggatccctcgagatggccgaggtgcagctggtgcagtctggagcagaggtgaaaaagcccggggagtctctgaagatctcctgtaagggttctggatacagctttaccagctactggatcggctgggtgcgccagatgcccgggaaaggcctggagtggatggggatcatctatcctggtgactctgataccagatacagcccgtccttccaaggccacgtcaccatctcagctgacaagtccatcagcactgcctacctgcagtggagcagcctgaaggcctcggacaccgccatgtattactgtgcgcgctactctggttctttcgataactggggtcaaggtactctggtgaccgtctcctcagcggccgcaattgaagttatgtatcctcctccttacctagacaatgagaagagcaatggaaccattatccatgtgaaagggaaacacctttgtccaagtcccctatttcccggaccttctaagcccttttgggtgctggtggtggttggtggagtcctggcttgctatagcttgctagtaacagtggcctttattattttctgggtgaggagtaagaggagcaggctcctgcacagtgactacatgaacatgactccccgccgccccgggcccacccgcaagcattaccagccctatgccccaccacgcgacttcgcagcctatcgctccagagtgaagttcagcaggagcgcagacgcccccgcgtaccagcagggccagaaccagctctataacgagctcaatctaggacgaagagaggagtacgatgttttggacaagagacgtggccgggaccctgagatggggggaaagccgagaaggaagaaccctcaggaaggcctgtacaatgaactgcagaaagataagatggcggaggcctacagtgagattgggatgaaaggcgagcgccggaggggcaaggggcacgatggcctttaccagggtctcagtacagccaccaaggacacctacgacgcccttcacatgcaggccctgccccctcgc

SEQ ID NO: 210 - protein, 15 aa, synthetic construct
  REGION 1..15: note = Description of Artificial Sequence: Synthetic peptide
GGGGSGGGGSGGGGS

SEQ ID NO: 211 - DNA, 45 bp, synthetic construct
  misc_feature 1..45: note = Description of Artificial Sequence: Synthetic oligonucleotide
  source 1..45: mol_type = other DNA
ggtggaggtggatcaggtggaggtggatctggtggaggtggatct

SEQ ID NO: 212 - protein, 5 aa, synthetic construct
  REGION 1..5: note = Description of Artificial Sequence: Synthetic peptide
GGGGS

SEQ ID NO: 213 - protein, 7 aa, synthetic construct
  REGION 1..7: note = Description of Artificial Sequence: Synthetic peptide
SGGSGGS

SEQ ID NO: 214 - protein, 9 aa, synthetic construct
  REGION 1..9: note = Description of Artificial Sequence: Synthetic peptide
GGGGSGGGS

SEQ ID NO: 215 - protein, 10 aa, synthetic construct
  REGION 1..10: note = Description of Artificial Sequence: Synthetic peptide
GGGGSGGGGS

SEQ ID NO: 216 - protein, 18 aa, synthetic construct
  REGION 1..18: note = Description of Artificial Sequence: Synthetic peptide
GGGGSGGGGSGGGGGGGS

SEQ ID NO: 217 - protein, 20 aa, synthetic construct
  REGION 1..20: note = Description of Artificial Sequence: Synthetic peptide
GGGGSGGGGSGGGGSGGGGS

SEQ ID NO: 218 - protein, 25 aa, synthetic construct
  REGION 1..25: note = Description of Artificial Sequence: Synthetic peptide
GGGGSGGGGSGGGGSGGGGSGGGGS

SEQ ID NO: 219 - protein, 30 aa, synthetic construct
  REGION 1..30: note = Description of Artificial Sequence: Synthetic polypeptide
GGGGSGGGGSGGGGSGGGGSGGGGSGGGGS

SEQ ID NO: 220 - protein, 35 aa, synthetic construct
  REGION 1..35: note = Description of Artificial Sequence: Synthetic polypeptide
GGGGSGGGGSGGGGSGGGGSGGGGSGGGGSGGGGS

SEQ ID NO: 221 - protein, 15 aa, synthetic construct
  REGION 1..15: note = Description of Artificial Sequence: Synthetic peptide
EPKSCDKTHTCPPCP

SEQ ID NO: 222 - protein, 24 aa, synthetic construct
  REGION 1..24: note = Description of Artificial Sequence: Synthetic peptide
GGGGSGGGSEPKSCDKTHTCPPCP

SEQ ID NO: 223 - protein, 62 aa, synthetic construct
  REGION 1..62: note = Description of Artificial Sequence: Synthetic polypeptide
ELKTPLGDTTHTCPRCPEPKSCDTPPPCPRCPEPKSCDTPPPCPRCPEPKSCDTPPPCPRCP

SEQ ID NO: 224 - protein, 6 aa, synthetic construct
  REGION 1..6: note = Description of Artificial Sequence: Synthetic peptide
GSGSGS

SEQ ID NO: 225 - skipped

SEQ ID NO: 226 - protein, 235 aa, Homo sapiens
MALPVTALLLPLALLLHAARPSQFRVSPLDRTWNLGETVELKCQVLLSNPTSGCSWLFQPRGAAASPTFLLYLSQNKPKAAEGLDTQRFSGKRLGDTFVLTLSDFRRENEGCYFCSALSNSIMYFSHFVPVFLPAKPTTTPAPRPPTPAPTIASQPLSLRPEACRPAAGGAVHTRGLDFACDIYIWAPLAGTCGVLLLSLVITLYCNHRNRRRVCKCPRPVVKSGDKPSLSARYV

SEQ ID NO: 227 - DNA, 213 bp, Homo sapiens
  source 1..213: mol_type = other DNA
cccaccacgacgccagcgccgcgaccaccaaccccggcgcccacgatcgcgtcgcagcccctgtccctgcgcccagaggcgtgccggccagcggcggggggcgcagtgcacacgagggggctggacttcgcctgtgatatctacatctgggcgcccctggccgggacttgtggggtccttctcctgtcactggttatcaccctttactgcaac

SEQ ID NO: 228 - DNA, 126 bp, Homo sapiens
  source 1..126: mol_type = other DNA
aaacggggcagaaagaagctcctgtatatattcaaacaaccatttatgagaccagtacaaactactcaagaggaagatggctgtagctgccgatttccagaagaagaagaaggaggatgtgaactg

SEQ ID NO: 229 - DNA, 7671 bp, synthetic construct
  misc_feature 1..7671: note = Description of Artificial Sequence: Synthetic polynucleotide
  source 1..7671: mol_type = other DNA
ccttctctaggcgcccccatatggccatatgagatcttatatggggcacccccgccccttgtaaacttccctgaccctgacatgacaagagttactaacagcccctctctccaagctcacttacaggctctctacttagtccagcacgaagtctggagacctctggcggcagcctaccaagaacaactggaccgaccggtgccgccaccatggaaaccgacaccctgctgctgtgggtgctgctgctgtgggtgccaggatccacaggactgcctgtgctgactcagccaccctcagcgtctgggacccccgggcagagggtcaccatctcttgttctggacgcagttccaacatcgggagtaattctgttaactggtatcgacaactcccaggagcggcccccaaactcctcatctatagtaataatcagcggcccccaggggtccctgtgcgattctctggctccaagtctggcacctcagcctccctggccatcagtgggctccagtctgaagatgaggccacttattactgtgcaacatgggatgacaatctgaatgttcactatgtcttcggaactgggaccaaggtcaccgtcctaggttctagaggtggtggtggtagcggcggcggcggctctggtggtggtggatccctcgagatggcccaggtgcagctggtgcagtctggggctgaggtgaagaagcctgggtcctcggtgaaggtctcctgcaaggcttctggaggcaccttcagcagctatgctatcagctgggtgcgacaggcccctggacaagggcttgagtggatgggaaggatcatccctatccttggtatagcaaactacgcacagaagttccagggcagagtcacgattaccgcggacaaatccacgagcacagcctacatggagctgagcagcctgagatctgaggacacggccgtgtattactgtgcgcgcggtggttactactctcatgacatgtggtctgaagattggggtcaaggtactctggtgaccgtctcctcagcggccgcacccaccacgacgccagcgccgcgaccaccaaccccggcgcccacgatcgcgtcgcagcccctgtccctgcgcccagaggcgtgccggccagcggcggggggcgcagtgcacacgagggggctggacttcgcctgtgatatctacatctgggcgcccctggccgggacttgtggggtccttctcctgtcactggttatcaccctttactgcaacaaacggggcagaaagaagctcctgtatatattcaaacaaccatttatgagaccagtacaaactactcaagaggaagatggctgtagctgccgatttccagaagaagaagaaggaggatgtgaactgagagtgaagttcagcaggagcgcagagccccccgcgtaccagcagggccagaaccagctctataacgagctcaatctaggacgaagagaggagtacgatgttttggacaagagacgtggccgggaccctgagatggggggaaagccgagaaggaagaaccctcaggaaggcctgtacaatgaactgcagaaagataagatggcggaggcctacagtgagattgggatgaaaggcgagcgccggaggggcaaggggcacgatggcctttaccagggtctcagtacagccaccaaggacacctacgacgcccttcacatgcaggccctgccccctcgctaacagccactcgaggatccggattagtccaatttgttaaagacaggatatcagtggtccaggctctagttttgactcaacaatatcaccagctgaagcctatagagtacgagccatagataaaataaaagattttatttagtctccagaaaaaggggggaatgaaagaccccacctgtaggtttggcaagctagcttaagtaacgccattttgcaaggcatggaaaaatacataactgagaatagagaagttcagatcaaggtcaggaacagatggaacagctgaatatgggccaaacaggatatctgtggtaagcagttcctgccccggctcagggccaagaacagatggaacagctgaatatgggccaaacaggatatctgtggtaagcagttcctgccccggctcagggccaagaacagatggtccccagatgcggtccagccctcagcagtttctagagaaccatcagatgtttccagggtgccccaaggacctgaaatgaccctgtgccttatttgaactaaccaatcagttcgcttctcgcttctgttcgcgcgcttctgctccccgagctcaataaaagagcccacaacccctcactcggggcgccagtcctccgattgactgagtcgcccgggtacccgtgtatccaataaaccctcttgcagttgcatccgacttgtggtctcgctgttccttgggagggtctcctctgagtgattgactacccgtcagcgggggtctttcacacatgcagcatgtatcaaaattaatttggttttttttcttaagtatttacattaaatggccatagtacttaaagttacattggcttccttgaaataaacatggagtattcagaatgtgtcataaatatttctaattttaagatagtatctccattggctttctactttttcttttatttttttttgtcctctgtcttccatttgttgttgttgttgtttgtttgtttgtttgttggttggttggttaatttttttttaaagatcctacactatagttcaagctagactattagctactctgtaacccagggtgaccttgaagtcatgggtagcctgctgttttagccttcccacatctaagattacaggtatgagctatcatttttggtatattgattgattgattgattgatgtgtgtgtgtgtgattgtgtttgtgtgtgtgactgtgaaaatgtgtgtatgggtgtgtgtgaatgtgtgtatgtatgtgtgtgtgtgagtgtgtgtgtgtgtgtgtgcatgtgtgtgtgtgtgactgtgtctatgtgtatgactgtgtgtgtgtgtgtgtgtgtgtgtgtgtgtgtgtgtgtgtgtgtgttgtgaaaaaatattctatggtagtgagagccaacgctccggctcaggtgtcaggttggtttttgagacagagtctttcacttagcttggaattcactggccgtcgttttacaacgtcgtgactgggaaaaccctggcgttacccaacttaatcgccttgcagcacatccccctttcgccagctggcgtaatagcgaagaggcccgcaccgatcgcccttcccaacagttgcgcagcctgaatggcgaatggcgcctgatgcggtattttctccttacgcatctgtgcggtatttcacaccgcatatggtgcactctcagtacaatctgctctgatgccgcatagttaagccagccccgacacccgccaacacccgctgacgcgccctgacgggcttgtctgctcccggcatccgcttacagacaagctgtgaccgtctccgggagctgcatgtgtcagaggttttcaccgtcatcaccgaaacgcgcgatgacgaaagggcctcgtgatacgcctatttttataggttaatgtcatgataataatggtttcttagacgtcaggtggcacttttcggggaaatgtgcgcggaacccctatttgtttatttttctaaatacattcaaatatgtatccgctcatgagacaataaccctgataaatgcttcaataatattgaaaaaggaagagtatgagtattcaacatttccgtgtcgcccttattcccttttttgcggcattttgccttcctgtttttgctcacccagaaacgctggtgaaagtaaaagatgctgaagatcagttgggtgcacgagtgggttacatcgaactggatctcaacagcggtaagatccttgagagttttcgccccgaagaacgttttccaatgatgagcacttttaaagttctgctatgtggcgcggtattatcccgtattgacgccgggcaagagcaactcggtcgccgcatacactattctcagaatgacttggttgagtactcaccagtcacagaaaagcatcttacggatggcatgacagtaagagaattatgcagtgctgccataaccatgagtgataacactgcggccaacttacttctgacaacgatcggaggaccgaaggagctaaccgcttttttgcacaacatgggggatcatgtaactcgccttgatcgttgggaaccggagctgaatgaagccataccaaacgacgagcgtgacaccacgatgcctgtagcaatggcaacaacgttgcgcaaactattaactggcgaactacttactctagcttcccggcaacaattaatagactggatggaggcggataaagttgcaggaccacttctgcgctcggcccttccggctggctggtttattgctgataaatctggagccggtgagcgtgggtctcgcggtatcattgcagcactggggccagatggtaagccctcccgtatcgtagttatctacacgacggggagtcaggcaactatggatgaacgaaatagacagatcgctgagataggtgcctcactgattaagcattggtaactgtcagaccaagtttactcatatatactttagattgatttaaaacttcatttttaatttaaaaggatctaggtgaagatcctttttgataatctcatgaccaaaatcccttaacgtgagttttcgttccactgagcgtcagaccccgtagaaaagatcaaaggatcttcttgagatcctttttttctgcgcgtaatctgctgcttgcaaacaaaaaaaccaccgctaccagcggtggtttgtttgccggatcaagagctaccaactctttttccgaaggtaactggcttcagcagagcgcagataccaaatactgtccttctagtgtagccgtagttaggccaccacttcaagaactctgtagcaccgcctacatacctcgctctgctaatcctgttaccagtggctgctgccagtggcgataagtcgtgtcttaccgggttggactcaagacgatagttaccggataaggcgcagcggtcgggctgaacggggggttcgtgcacacagcccagcttggagcgaacgacctacaccgaactgagatacctacagcgtgagcattgagaaagcgccacgcttcccgaagggagaaaggcggacaggtatccggtaagcggcagggtcggaacaggagagcgcacgagggagcttccagggggaaacgcctggtatctttatagtcctgtcgggtttcgccacctctgacttgagcgtcgatttttgtgatgctcgtcaggggggcggagcctatggaaaaacgccagcaacgcggcctttttacggttcctggccttttgctggccttttgctcacatgttctttcctgcgttatcccctgattctgtggataaccgtattaccgcctttgagtgagctgataccgctcgccgcagccgaacgaccgagcgcagcgagtcagtgagcgaggaagcggaagagcgcccaatacgcaaaccgcctctccccgcgcgttggccgattcattaatgcagctggcacgacaggtttcccgactggaaagcgggcagtgagcgcaacgcaattaatgtgagttagctcactcattaggcaccccaggctttacactttatgcttccggctcgtatgttgtgtggaattgtgagcggataacaatttcacacaggaaacagctatgaccatgattacgccaagctttgctcttaggagtttcctaatacatcccaaactcaaatatataaagcatttgacttgttctatgccctagggggcggggggaagctaagccagctttttttaacatttaaaatgttaattccattttaaatgcacagatgtttttatttcataagggtttcaatgtgcatgaatgctgcaatattcctgttaccaaagctagtataaataaaaatagataaacgtggaaattacttagagtttctgtcattaacgtttccttcctcagttgacaacataaatgcgctgctgagcaagccagtttgcatctgtcaggatcaatttcccattatgccagtcatattaattactagtcaattagttgatttttatttttgacatatacatgtgaatgaaagaccccacctgtaggtttggcaagctagcttaagtaacgccattttgcaaggcatggaaaaatacataactgagaatagaaaagttcagatcaaggtcaggaacagatggaacagctgaatatgggccaaacaggatatctgtggtaagcagttcctgccccggctcagggccaagaacagatggaacagctgaatatgggccaaacaggatatctgtggtaagcagttcctgccccggctcagggccaagaacagatggtccccagatgcggtccagccctcagcagtttctagagaaccatcagatgtttccagggtgccccaaggacctgaaatgaccctgtgccttatttgaactaaccaatcagttcgcttctcgcttctgttcgcgcgcttatgctccccgagctcaataaaagagcccacaacccctcactcggggcgccagtcctccgattgactgagtcgcccgggtacccgtgtatccaataaaccctcttgcagttgcatccgacttgtggtctcgctgttccttgggagggtctcctctgagtgattgactacccgtcagcgggggtctttcatttgggggctcgtccgggatcgggagacccctgcccagggaccaccgacccaccaccgggaggtaagctggccagcaacttatctgtgtctgtccgattgtctagtgtctatgactgattttatgcgcctgcgtcggtactagttagctaactagctctgtatctggcggacccgtggtggaactgacgagttcggaacacccggccgcaaccctgggagacgtcccagggacttcgggggccgtttttgtggcccgacctgagtcctaaaatcccgatcgtttaggactctttggtgcaccccccttagaggagggatatgtggttctggtaggagacgagaacctaaaacagttcccgcctccgtctgaatttttgctttcggtttgggaccgaagccgcgccgcgcgtcttgtctgctgcagcatcgttctgtgttgtctctgtctgactgtgtttctgtatttgtctgaaaatatgggcccgggctagactgttaccactcccttaagtttgaccttaggtcactggaaagatgtcgagcggatcgctcacaaccagtcggtagatgtcaagaagagacgttgggttaccttctgctctgcagaatggccaacctttaacgtcggatggccgcgagacggcacctttaaccgagacctcatcacccaggttaagatcaaggtcttttcacctggcccgcatggacacccagaccaggtcccctacatcgtgacctgggaagccttggcttttgacccccctccctgggtcaagccctttgtacaccctaagcctccgcctcctcttcctccatccgccccgtctctcccccttgaacctcctcgttcgaccccgcctcgatcctccctttatccagccctcact

SEQ ID NO: 230 - DNA, 7653 bp, synthetic construct
  misc_feature 1..7653: note = Description of Artificial Sequence: Synthetic polynucleotide
  source 1..7653: mol_type = other DNA
ggccctctaggcgcccccatatggccatatgagatcttatatggggcacccccgccccttgtaaacttccctgaccctgacatgacaagagttactaacagcccctctctccaagctcacttacaggctctctacttagtccagcacgaagtctggagacctctggcggcagcctaccaagaacaactggaccgaccggtgccgccaccatggaaaccgacaccctgctgctgtgggtgctgctgctgtgggtgccaggatccacaggatcctatgagctgactcagccaccctcagcgtctgggacccccgggcagagggtcaccatgtcttgttctggaaccagctccaacatcggaagtcactctgtaaactggtaccagcagctcccaggaacggcccccaaactcctcatctatactaataatcagcggccctcaggggtccctgaccgattctctggctccaagtctggcacctcagcctccctggccatcagtggcctccagtctgaggatgaggctgattattactgtgcagcatgggatggcagcctgaatggtctggtattcggcggagggaccaagctgaccgtcctaggttctagaggtggtggtggtagcggcggcggcggctctggtggtggtggatccctcgagatggccgaggtgcagctggtgcagtctggagcagaggtgaaaaagcccggggagtctctgaagatctcctgtaagggttctggatacagctttaccagctactggatcggctgggtgcgccagatgcccgggaaaggcctggagtggatggggatcatctatcctggtgactctgataccagatacagcccgtccttccaaggccacgtcaccatctcagctgacaagtccatcagcactgcctacctgcagtggagcagcctgaaggcctcggacaccgccatgtattactgtgcgcgctactctggttctttcgataactggggtcaaggtactctggtgaccgtctcctcagcggccgcacccaccacgacgccagcgccgcgaccaccaaccccggcgcccacgatcgcgtcgcagcccctgtccctgcgcccagaggcgtgccggccagcggcggggggcgcagtgcacacgagggggctggacttcgcctgtgatatctacatctgggcgcccctggccgggacttgtggggtccttctcctgtcactggttatcaccctttactgcaacaaacggggcagaaagaagctcctgtatatattcaaacaaccatttatgagaccagtacaaactactcaagaggaagatggctgtagctgccgatttccagaagaagaagaaggaggatgtgaactgagagtgaagttcagcaggagcgcagagccccccgcgtaccagcagggccagaaccagctctataacgagctcaatctaggacgaagagaggagtacgatgttttggacaagagacgtggccgggaccctgagatggggggaaagccgagaaggaagaaccctcaggaaggcctgtacaatgaactgcagaaagataagatggcggaggcctacagtgagattgggatgaaaggcgagcgccggaggggcaaggggcacgatggcctttaccagggtctcagtacagccaccaaggacacctacgacgcccttcacatgcaggccctgccccctcgctaacagccactcgaggatccggattagtccaatttgttaaagacaggatatcagtggtccaggctctagttttgactcaacaatatcaccagctgaagcctatagagtacgagccatagataaaataaaagattttatttagtctccagaaaaaggggggaatgaaagaccccacctgtaggtttggcaagctagcttaagtaacgccattttgcaaggcatggaaaaatacataactgagaatagagaagttcagatcaaggtcaggaacagatggaacagctgaatatgggccaaacaggatatctgtggtaagcagttcctgccccggctcagggccaagaacagatggaacagctgaatatgggccaaacaggatatctgtggtaagcagttcctgccccggctcagggccaagaacagatggtccccagatgcggtccagccctcagcagtttctagagaaccatcagatgtttccagggtgccccaaggacctgaaatgaccctgtgccttatttgaactaaccaatcagttcgcttctcgcttctgttcgcgcgcttctgctccccgagctcaataaaagagcccacaacccctcactcggggcgccagtcctccgattgactgagtcgcccgggtacccgtgtatccaataaaccctcttgcagttgcatccgacttgtggtctcgctgttccttgggagggtctcctctgagtgattgactacccgtcagcgggggtctttcacacatgcagcatgtatcaaaattaatttggttttttttcttaagtatttacattaaatggccatagtacttaaagttacattggcttccttgaaataaacatggagtattcagaatgtgtcataaatatttctaattttaagatagtatctccattggctttctactttttcttttatttttttttgtcctctgtcttccatttgttgttgttgttgtttgtttgtttgtttgttggttggttggttaatttttttttaaagatcctacactatagttcaagctagactattagctactctgtaacccagggtgaccttgaagtcatgggtagcctgctgttttagccttcccacatctaagattacaggtatgagctatcatttttggtatattgattgattgattgattgatgtgtgtgtgtgtgattgtgtttgtgtgtgtgactgtgaaaatgtgtgtatgggtgtgtgtgaatgtgtgtatgtatgtgtgtgtgtgagtgtgtgtgtgtgtgtgtgcatgtgtgtgtgtgtgactgtgtctatgtgtatgactgtgtgtgtgtgtgtgtgtgtgtgtgtgtgtgtgtgtgtgtgtgtgttgtgaaaaaatattctatggtagtgagagccaacgctccggctcaggtgtcaggttggtttttgagacagagtctttcacttagcttggaattcactggccgtcgttttacaacgtcgtgactgggaaaaccctggcgttacccaacttaatcgccttgcagcacatccccctttcgccagctggcgtaatagcgaagaggcccgcaccgatcgcccttcccaacagttgcgcagcctgaatggcgaatggcgcctgatgcggtattttctccttacgcatctgtgcggtatttcacaccgcatatggtgcactctcagtacaatctgctctgatgccgcatagttaagccagccccgacacccgccaacacccgctgacgcgccctgacgggcttgtctgctcccggcatccgcttacagacaagctgtgaccgtctccgggagctgcatgtgtcagaggttttcaccgtcatcaccgaaacgcgcgatgacgaaagggcctcgtgatacgcctatttttataggttaatgtcatgataataatggtttcttagacgtcaggtggcacttttcggggaaatgtgcgcggaacccctatttgtttatttttctaaatacattcaaatatgtatccgctcatgagacaataaccctgataaatgcttcaataatattgaaaaaggaagagtatgagtattcaacatttccgtgtcgcccttattcccttttttgcggcattttgccttcctgtttttgctcacccagaaacgctggtgaaagtaaaagatgctgaagatcagttgggtgcacgagtgggttacatcgaactggatctcaacagcggtaagatccttgagagttttcgccccgaagaacgttttccaatgatgagcacttttaaagttctgctatgtggcgcggtattatcccgtattgacgccgggcaagagcaactcggtcgccgcatacactattctcagaatgacttggttgagtactcaccagtcacagaaaagcatcttacggatggcatgacagtaagagaattatgcagtgctgccataaccatgagtgataacactgcggccaacttacttctgacaacgatcggaggaccgaaggagctaaccgcttttttgcacaacatgggggatcatgtaactcgccttgatcgttgggaaccggagctgaatgaagccataccaaacgacgagcgtgacaccacgatgcctgtagcaatggcaacaacgttgcgcaaactattaactggcgaactacttactctagcttcccggcaacaattaatagactggatggaggcggataaagttgcaggaccacttctgcgctcggcccttccggctggctggtttattgctgataaatctggagccggtgagcgtgggtctcgcggtatcattgcagcactggggccagatggtaagccctcccgtatcgtagttatctacacgacggggagtcaggcaactatggatgaacgaaatagacagatcgctgagataggtgcctcactgattaagcattggtaactgtcagaccaagtttactcatatatactttagattgatttaaaacttcatttttaatttaaaaggatctaggtgaagatcctttttgataatctcatgaccaaaatcccttaacgtgagttttcgttccactgagcgtcagaccccgtagaaaagatcaaaggatcttcttgagatcctttttttctgcgcgtaatctgctgcttgcaaacaaaaaaaccaccgctaccagcggtggtttgtttgccggatcaagagctaccaactctttttccgaaggtaactggcttcagcagagcgcagataccaaatactgtccttctagtgtagccgtagttaggccaccacttcaagaactctgtagcaccgcctacatacctcgctctgctaatcctgttaccagtggctgctgccagtggcgataagtcgtgtcttaccgggttggactcaagacgatagttaccggataaggcgcagcggtcgggctgaacggggggttcgtgcacacagcccagcttggagcgaacgacctacaccgaactgagatacctacagcgtgagcattgagaaagcgccacgcttcccgaagggagaaaggcggacaggtatccggtaagcggcagggtcggaacaggagagcgcacgagggagcttccagggggaaacgcctggtatctttatagtcctgtcgggtttcgccacctctgacttgagcgtcgatttttgtgatgctcgtcaggggggcggagcctatggaaaaacgccagcaacgcggcctttttacggttcctggccttttgctggccttttgctcacatgttctttcctgcgttatcccctgattctgtggataaccgtattaccgcctttgagtgagctgataccgctcgccgcagccgaacgaccgagcgcagcgagtcagtgagcgaggaagcggaagagcgcccaatacgcaaaccgcctctccccgcgcgttggccgattcattaatgcagctggcacgacaggtttcccgactggaaagcgggcagtgagcgcaacgcaattaatgtgagttagctcactcattaggcaccccaggctttacactttatgcttccggctcgtatgttgtgtggaattgtgagcggataacaatttcacacaggaaacagctatgaccatgattacgccaagctttgctcttaggagtttcctaatacatcccaaactcaaatatataaagcatttgacttgttctatgccctagggggcggggggaagctaagccagctttttttaacatttaaaatgttaattccattttaaatgcacagatgtttttatttcataagggtttcaatgtgcatgaatgctgcaatattcctgttaccaaagctagtataaataaaaatagataaacgtggaaattacttagagtttctgtcattaacgtttccttcctcagttgacaacataaatgcgctgctgagcaagccagtttgcatctgtcaggatcaatttcccattatgccagtcatattaattactagtcaattagttgatttttatttttgacatatacatgtgaatgaaagaccccacctgtaggtttggcaagctagcttaagtaacgccattttgcaaggcatggaaaaatacataactgagaatagaaaagttcagatcaaggtcaggaacagatggaacagctgaatatgggccaaacaggatatctgtggtaagcagttcctgccccggctcagggccaagaacagatggaacagctgaatatgggccaaacaggatatctgtggtaagcagttcctgccccggctcagggccaagaacagatggtccccagatgcggtccagccctcagcagtttctagagaaccatcagatgtttccagggtgccccaaggacctgaaatgaccctgtgccttatttgaactaaccaatcagttcgcttctcgcttctgttcgcgcgcttatgctccccgagctcaataaaagagcccacaacccctcactcggggcgccagtcctccgattgactgagtcgcccgggtacccgtgtatccaataaaccctcttgcagttgcatccgacttgtggtctcgctgttccttgggagggtctcctctgagtgattgactacccgtcagcgggggtctttcatttgggggctcgtccgggatcgggagacccctgcccagggaccaccgacccaccaccgggaggtaagctggccagcaacttatctgtgtctgtccgattgtctagtgtctatgactgattttatgcgcctgcgtcggtactagttagctaactagctctgtatctggcggacccgtggtggaactgacgagttcggaacacccggccgcaaccctgggagacgtcccagggacttcgggggccgtttttgtggcccgacctgagtcctaaaatcccgatcgtttaggactctttggtgcaccccccttagaggagggatatgtggttctggtaggagacgagaacctaaaacagttcccgcctccgtctgaatttttgctttcggtttgggaccgaagccgcgccgcgcgtcttgtctgctgcagcatcgttctgtgttgtctctgtctgactgtgtttctgtatttgtctgaaaatatgggcccgggctagactgttaccactcccttaagtttgaccttaggtcactggaaagatgtcgagcggatcgctcacaaccagtcggtagatgtcaagaagagacgttgggttaccttctgctctgcagaatggccaacctttaacgtcggatggccgcgagacggcacctttaaccgagacctcatcacccaggttaagatcaaggtcttttcacctggcccgcatggacacccagaccaggtcccctacatcgtgacctgggaagccttggcttttgacccccctccctgggtcaagccctttgtacaccctaagcctccgcctcctcttcctccatccgccccgtctctcccccttgaacctcctcgttcgaccccgcctcgatcctccctttatccagccctcact

SEQ ID NO: 231 - DNA, 7668 bp, synthetic construct
  misc_feature 1..7668: note = Description of Artificial Sequence: Synthetic polynucleotide
  source 1..7668: mol_type = other DNA
ccttctctaggcgcccccatatggccatatgagatcttatatggggcacccccgccccttgtaaacttccctgaccctgacatgacaagagttactaacagcccctctctccaagctcacttacaggctctctacttagtccagcacgaagtctggagacctctggcggcagcctaccaagaacaactggaccgaccggtgccgccaccatggaaaccgacaccctgctgctgtgggtgctgctgctgtgggtgccaggatccacaggacaggctgtgctgactcagccaccctcagcgtctgggacccccgggcagagggtcaccatctcttgttctggaagcagctccaacatcggaagtaattacgtattctggtaccagcagctcccaggaacggcccccaaactcctcatctatagtaataatcagcggccctcaggggtccctgaccgattctctggctccaagtctggcacctcagcctccctggccatcagtgggctccggtccgaggatgaggctgattattactgtgcagcatgggatgacagcctgagtgcctcttatgttttcggaactgggaccaaggtcaccgtcctaggttctagaggtggtggtggtagcggcggcggcggctctggtggtggtggatccctcgagatggcccaggtgcagctggtgcagtctggggctgaggtgaagaagcctgggtcctcggtgaaggtctcctgcaaggcttctggaggcaccttcagcagctatgctatcagctgggtgcgacaggcccctggacaagggcttgagtggatgggaaggatcatccctatccttggtacagcaaactacgcacagaagttccagggcagagtcacgattaccgcggacgaatccacgagcacagcctacatggagctgagcagcctgagatctgaggacacggccgtgtattactgtgcgcgctctggttacggttcttaccgttgggaagattcttggggtcaaggtactctggtgaccgtctcctcagcggccgcacccaccacgacgccagcgccgcgaccaccaaccccggcgcccacgatcgcgtcgcagcccctgtccctgcgcccagaggcgtgccggccagcggcggggggcgcagtgcacacgagggggctggacttcgcctgtgatatctacatctgggcgcccctggccgggacttgtggggtccttctcctgtcactggttatcaccctttactgcaacaaacggggcagaaagaagctcctgtatatattcaaacaaccatttatgagaccagtacaaactactcaagaggaagatggctgtagctgccgatttccagaagaagaagaaggaggatgtgaactgagagtgaagttcagcaggagcgcagagccccccgcgtaccagcagggccagaaccagctctataacgagctcaatctaggacgaagagaggagtacgatgttttggacaagagacgtggccgggaccctgagatggggggaaagccgagaaggaagaaccctcaggaaggcctgtacaatgaactgcagaaagataagatggcggaggcctacagtgagattgggatgaaaggcgagcgccggaggggcaaggggcacgatggcctttaccagggtctcagtacagccaccaaggacacctacgacgcccttcacatgcaggccctgccccctcgctaacagccactcgaggatccggattagtccaatttgttaaagacaggatatcagtggtccaggctctagttttgactcaacaatatcaccagctgaagcctatagagtacgagccatagataaaataaaagattttatttagtctccagaaaaaggggggaatgaaagaccccacctgtaggtttggcaagctagcttaagtaacgccattttgcaaggcatggaaaaatacataactgagaatagagaagttcagatcaaggtcaggaacagatggaacagctgaatatgggccaaacaggatatctgtggtaagcagttcctgccccggctcagggccaagaacagatggaacagctgaatatgggccaaacaggatatctgtggtaagcagttcctgccccggctcagggccaagaacagatggtccccagatgcggtccagccctcagcagtttctagagaaccatcagatgtttccagggtgccccaaggacctgaaatgaccctgtgccttatttgaactaaccaatcagttcgcttctcgcttctgttcgcgcgcttctgctccccgagctcaataaaagagcccacaacccctcactcggggcgccagtcctccgattgactgagtcgcccgggtacccgtgtatccaataaaccctcttgcagttgcatccgacttgtggtctcgctgttccttgggagggtctcctctgagtgattgactacccgtcagcgggggtctttcacacatgcagcatgtatcaaaattaatttggttttttttcttaagtatttacattaaatggccatagtacttaaagttacattggcttccttgaaataaacatggagtattcagaatgtgtcataaatatttctaattttaagatagtatctccattggctttctactttttcttttatttttttttgtcctctgtcttccatttgttgttgttgttgtttgtttgtttgtttgttggttggttggttaatttttttttaaagatcctacactatagttcaagctagactattagctactctgtaacccagggtgaccttgaagtcatgggtagcctgctgttttagccttcccacatctaagattacaggtatgagctatcatttttggtatattgattgattgattgattgatgtgtgtgtgtgtgattgtgtttgtgtgtgtgactgtgaaaatgtgtgtatgggtgtgtgtgaatgtgtgtatgtatgtgtgtgtgtgagtgtgtgtgtgtgtgtgtgcatgtgtgtgtgtgtgactgtgtctatgtgtatgactgtgtgtgtgtgtgtgtgtgtgtgtgtgtgtgtgtgtgtgtgtgtgttgtgaaaaaatattctatggtagtgagagccaacgctccggctcaggtgtcaggttggtttttgagacagagtctttcacttagcttggaattcactggccgtcgttttacaacgtcgtgactgggaaaaccctggcgttacccaacttaatcgccttgcagcacatccccctttcgccagctggcgtaatagcgaagaggcccgcaccgatcgcccttcccaacagttgcgcagcctgaatggcgaatggcgcctgatgcggtattttctccttacgcatctgtgcggtatttcacaccgcatatggtgcactctcagtacaatctgctctgatgccgcatagttaagccagccccgacacccgccaacacccgctgacgcgccctgacgggcttgtctgctcccggcatccgcttacagacaagctgtgaccgtctccgggagctgcatgtgtcagaggttttcaccgtcatcaccgaaacgcgcgatgacgaaagggcctcgtgatacgcctatttttataggttaatgtcatgataataatggtttcttagacgtcaggtggcacttttcggggaaatgtgcgcggaacccctatttgtttatttttctaaatacattcaaatatgtatccgctcatgagacaataaccctgataaatgcttcaataatattgaaaaaggaagagtatgagtattcaacatttccgtgtcgcccttattcccttttttgcggcattttgccttcctgtttttgctcacccagaaacgctggtgaaagtaaaagatgctgaagatcagttgggtgcacgagtgggttacatcgaactggatctcaacagcggtaagatccttgagagttttcgccccgaagaacgttttccaatgatgagcacttttaaagttctgctatgtggcgcggtattatcccgtattgacgccgggcaagagcaactcggtcgccgcatacactattctcagaatgacttggttgagtactcaccagtcacagaaaagcatcttacggatggcatgacagtaagagaattatgcagtgctgccataaccatgagtgataacactgcggccaacttacttctgacaacgatcggaggaccgaaggagctaaccgcttttttgcacaacatgggggatcatgtaactcgccttgatcgttgggaaccggagctgaatgaagccataccaaacgacgagcgtgacaccacgatgcctgtagcaatggcaacaacgttgcgcaaactattaactggcgaactacttactctagcttcccggcaacaattaatagactggatggaggcggataaagttgcaggaccacttctgcgctcggcccttccggctggctggtttattgctgataaatctggagccggtgagcgtgggtctcgcggtatcattgcagcactggggccagatggtaagccctcccgtatcgtagttatctacacgacggggagtcaggcaactatggatgaacgaaatagacagatcgctgagataggtgcctcactgattaagcattggtaactgtcagaccaagtttactcatatatactttagattgatttaaaacttcatttttaatttaaaaggatctaggtgaagatcctttttgataatctcatgaccaaaatcccttaacgtgagttttcgttccactgagcgtcagaccccgtagaaaagatcaaaggatcttcttgagatcctttttttctgcgcgtaatctgctgcttgcaaacaaaaaaaccaccgctaccagcggtggtttgtttgccggatcaagagctaccaactctttttccgaaggtaactggcttcagcagagcgcagataccaaatactgtccttctagtgtagccgtagttaggccaccacttcaagaactctgtagcaccgcctacatacctcgctctgctaatcctgttaccagtggctgctgccagtggcgataagtcgtgtcttaccgggttggactcaagacgatagttaccggataaggcgcagcggtcgggctgaacggggggttcgtgcacacagcccagcttggagcgaacgacctacaccgaactgagatacctacagcgtgagcattgagaaagcgccacgcttcccgaagggagaaaggcggacaggtatccggtaagcggcagggtcggaacaggagagcgcacgagggagcttccagggggaaacgcctggtatctttatagtcctgtcgggtttcgccacctctgacttgagcgtcgatttttgtgatgctcgtcaggggggcggagcctatggaaaaacgccagcaacgcggcctttttacggttcctggccttttgctggccttttgctcacatgttctttcctgcgttatcccctgattctgtggataaccgtattaccgcctttgagtgagctgataccgctcgccgcagccgaacgaccgagcgcagcgagtcagtgagcgaggaagcggaagagcgcccaatacgcaaaccgcctctccccgcgcgttggccgattcattaatgcagctggcacgacaggtttcccgactggaaagcgggcagtgagcgcaacgcaattaatgtgagttagctcactcattaggcaccccaggctttacactttatgcttccggctcgtatgttgtgtggaattgtgagcggataacaatttcacacaggaaacagctatgaccatgattacgccaagctttgctcttaggagtttcctaatacatcccaaactcaaatatataaagcatttgacttgttctatgccctagggggcggggggaagctaagccagctttttttaacatttaaaatgttaattccattttaaatgcacagatgtttttatttcataagggtttcaatgtgcatgaatgctgcaatattcctgttaccaaagctagtataaataaaaatagataaacgtggaaattacttagagtttctgtcattaacgtttccttcctcagttgacaacataaatgcgctgctgagcaagccagtttgcatctgtcaggatcaatttcccattatgccagtcatattaattactagtcaattagttgatttttatttttgacatatacatgtgaatgaaagaccccacctgtaggtttggcaagctagcttaagtaacgccattttgcaaggcatggaaaaatacataactgagaatagaaaagttcagatcaaggtcaggaacagatggaacagctgaatatgggccaaacaggatatctgtggtaagcagttcctgccccggctcagggccaagaacagatggaacagctgaatatgggccaaacaggatatctgtggtaagcagttcctgccccggctcagggccaagaacagatggtccccagatgcggtccagccctcagcagtttctagagaaccatcagatgtttccagggtgccccaaggacctgaaatgaccctgtgccttatttgaactaaccaatcagttcgcttctcgcttctgttcgcgcgcttatgctccccgagctcaataaaagagcccacaacccctcactcggggcgccagtcctccgattgactgagtcgcccgggtacccgtgtatccaataaaccctcttgcagttgcatccgacttgtggtctcgctgttccttgggagggtctcctctgagtgattgactacccgtcagcgggggtctttcatttgggggctcgtccgggatcgggagacccctgcccagggaccaccgacccaccaccgggaggtaagctggccagcaacttatctgtgtctgtccgattgtctagtgtctatgactgattttatgcgcctgcgtcggtactagttagctaactagctctgtatctggcggacccgtggtggaactgacgagttcggaacacccggccgcaaccctgggagacgtcccagggacttcgggggccgtttttgtggcccgacctgagtcctaaaatcccgatcgtttaggactctttggtgcaccccccttagaggagggatatgtggttctggtaggagacgagaacctaaaacagttcccgcctccgtctgaatttttgctttcggtttgggaccgaagccgcgccgcgcgtcttgtctgctgcagcatcgttctgtgttgtctctgtctgactgtgtttctgtatttgtctgaaaatatgggcccgggctagactgttaccactcccttaagtttgaccttaggtcactggaaagatgtcgagcggatcgctcacaaccagtcggtagatgtcaagaagagacgttgggttaccttctgctctgcagaatggccaacctttaacgtcggatggccgcgagacggcacctttaaccgagacctcatcacccaggttaagatcaaggtcttttcacctggcccgcatggacacccagaccaggtcccctacatcgtgacctgggaagccttggcttttgacccccctccctgggtcaagccctttgtacaccctaagcctccgcctcctcttcctccatccgccccgtctctcccccttgaacctcctcgttcgaccccgcctcgatcctccctttatccagccctcact

SEQ ID NO: 232 - DNA, 7662 bp, synthetic construct
  misc_feature 1..7662: note = Description of Artificial Sequence: Synthetic polynucleotide
  source 1..7662: mol_type = other DNA
ccttctctaggcgcccccatatggccatatgagatcttatatggggcacccccgccccttgtaaacttccctgaccctgacatgacaagagttactaacagcccctctctccaagctcacttacaggctctctacttagtccagcacgaagtctggagacctctggcggcagcctaccaagaacaactggaccgaccggtgccgccaccatggaaaccgacaccctgctgctgtgggtgctgctgctgtgggtgccaggatccacaggacagtctgtgctgacgcagccgccctcagtgtctggggccccagggcagagggtcaccatctcctgcactgggagcagctccaacatcggggcaggttttgatgtacactggtaccagcagcttccaggaacagcccccaaactcctcatctatggtaacagcaatcggccctcaggggtccctgaccgattctctggctccaagtctggcacctcagcctccctggccatcactgggctccaggctgaggatgaggctgattattactgccagtcctatgacagcagcctgagtggttatgtcttcggaactgggaccaaggtcaccgtcctaggttctagaggtggtggtggtagcggcggcggcggctctggtggtggtggatccctcgagatggcccaggtccagctggtacagtctggggctgaggtgaagaagcctggggcctcagtgaaggtctcctgcaaggcttctggatacaccttcaccgactactatatgcactgggtgcgacaggcccctggacaacggcttgagtggatgggatggatcaaccctaacagtggtggcacaaactatgcacagaagtttcaggacaggatcaccgtgaccagggacacctccagcaacacaggctacatggagctgaccaggctgagatctgacgacacggccgtgtattactgtgcgcgctctccgtactctggtgttctggataaatggggtcaaggtactctggtgaccgtctcctcagcggccgcacccaccacgacgccagcgccgcgaccaccaaccccggcgcccacgatcgcgtcgcagcccctgtccctgcgcccagaggcgtgccggccagcggcggggggcgcagtgcacacgagggggctggacttcgcctgtgatatctacatctgggcgcccctggccgggacttgtggggtccttctcctgtcactggttatcaccctttactgcaacaaacggggcagaaagaagctcctgtatatattcaaacaaccatttatgagaccagtacaaactactcaagaggaagatggctgtagctgccgatttccagaagaagaagaaggaggatgtgaactgagagtgaagttcagcaggagcgcagagccccccgcgtaccagcagggccagaaccagctctataacgagctcaatctaggacgaagagaggagtacgatgttttggacaagagacgtggccgggaccctgagatggggggaaagccgagaaggaagaaccctcaggaaggcctgtacaatgaactgcagaaagataagatggcggaggcctacagtgagattgggatgaaaggcgagcgccggaggggcaaggggcacgatggcctttaccagggtctcagtacagccaccaaggacacctacgacgcccttcacatgcaggccctgccccctcgctaacagccactcgaggatccggattagtccaatttgttaaagacaggatatcagtggtccaggctctagttttgactcaacaatatcaccagctgaagcctatagagtacgagccatagataaaataaaagattttatttagtctccagaaaaaggggggaatgaaagaccccacctgtaggtttggcaagctagcttaagtaacgccattttgcaaggcatggaaaaatacataactgagaatagagaagttcagatcaaggtcaggaacagatggaacagctgaatatgggccaaacaggatatctgtggtaagcagttcctgccccggctcagggccaagaacagatggaacagctgaatatgggccaaacaggatatctgtggtaagcagttcctgccccggctcagggccaagaacagatggtccccagatgcggtccagccctcagcagtttctagagaaccatcagatgtttccagggtgccccaaggacctgaaatgaccctgtgccttatttgaactaaccaatcagttcgcttctcgcttctgttcgcgcgcttctgctccccgagctcaataaaagagcccacaacccctcactcggggcgccagtcctccgattgactgagtcgcccgggtacccgtgtatccaataaaccctcttgcagttgcatccgacttgtggtctcgctgttccttgggagggtctcctctgagtgattgactacccgtcagcgggggtctttcacacatgcagcatgtatcaaaattaatttggttttttttcttaagtatttacattaaatggccatagtacttaaagttacattggcttccttgaaataaacatggagtattcagaatgtgtcataaatatttctaattttaagatagtatctccattggctttctactttttcttttatttttttttgtcctctgtcttccatttgttgttgttgttgtttgtttgtttgtttgttggttggttggttaatttttttttaaagatcctacactatagttcaagctagactattagctactctgtaacccagggtgaccttgaagtcatgggtagcctgctgttttagccttcccacatctaagattacaggtatgagctatcatttttggtatattgattgattgattgattgatgtgtgtgtgtgtgattgtgtttgtgtgtgtgactgtgaaaatgtgtgtatgggtgtgtgtgaatgtgtgtatgtatgtgtgtgtgtgagtgtgtgtgtgtgtgtgtgcatgtgtgtgtgtgtgactgtgtctatgtgtatgactgtgtgtgtgtgtgtgtgtgtgtgtgtgtgtgtgtgtgtgtgtgtgttgtgaaaaaatattctatggtagtgagagccaacgctccggctcaggtgtcaggttggtttttgagacagagtctttcacttagcttggaattcactggccgtcgttttacaacgtcgtgactgggaaaaccctggcgttacccaacttaatcgccttgcagcacatccccctttcgccagctggcgtaatagcgaagaggcccgcaccgatcgcccttcccaacagttgcgcagcctgaatggcgaatggcgcctgatgcggtattttctccttacgcatctgtgcggtatttcacaccgcatatggtgcactctcagtacaatctgctctgatgccgcatagttaagccagccccgacacccgccaacacccgctgacgcgccctgacgggcttgtctgctcccggcatccgcttacagacaagctgtgaccgtctccgggagctgcatgtgtcagaggttttcaccgtcatcaccgaaacgcgcgatgacgaaagggcctcgtgatacgcctatttttataggttaatgtcatgataataatggtttcttagacgtcaggtggcacttttcggggaaatgtgcgcggaacccctatttgtttatttttctaaatacattcaaatatgtatccgctcatgagacaataaccctgataaatgcttcaataatattgaaaaaggaagagtatgagtattcaacatttccgtgtcgcccttattcccttttttgcggcattttgccttcctgtttttgctcacccagaaacgctggtgaaagtaaaagatgctgaagatcagttgggtgcacgagtgggttacatcgaactggatctcaacagcggtaagatccttgagagttttcgccccgaagaacgttttccaatgatgagcacttttaaagttctgctatgtggcgcggtattatcccgtattgacgccgggcaagagcaactcggtcgccgcatacactattctcagaatgacttggttgagtactcaccagtcacagaaaagcatcttacggatggcatgacagtaagagaattatgcagtgctgccataaccatgagtgataacactgcggccaacttacttctgacaacgatcggaggaccgaaggagctaaccgcttttttgcacaacatgggggatcatgtaactcgccttgatcgttgggaaccggagctgaatgaagccataccaaacgacgagcgtgacaccacgatgcctgtagcaatggcaacaacgttgcgcaaactattaactggcgaactacttactctagcttcccggcaacaattaatagactggatggaggcggataaagttgcaggaccacttctgcgctcggcccttccggctggctggtttattgctgataaatctggagccggtgagcgtgggtctcgcggtatcattgcagcactggggccagatggtaagccctcccgtatcgtagttatctacacgacggggagtcaggcaactatggatgaacgaaatagacagatcgctgagataggtgcctcactgattaagcattggtaactgtcagaccaagtttactcatatatactttagattgatttaaaacttcatttttaatttaaaaggatctaggtgaagatcctttttgataatctcatgaccaaaatcccttaacgtgagttttcgttccactgagcgtcagaccccgtagaaaagatcaaaggatcttcttgagatcctttttttctgcgcgtaatctgctgcttgcaaacaaaaaaaccaccgctaccagcggtggtttgtttgccggatcaagagctaccaactctttttccgaaggtaactggcttcagcagagcgcagataccaaatactgtccttctagtgtagccgtagttaggccaccacttcaagaactctgtagcaccgcctacatacctcgctctgctaatcctgttaccagtggctgctgccagtggcgataagtcgtgtcttaccgggttggactcaagacgatagttaccggataaggcgcagcggtcgggctgaacggggggttcgtgcacacagcccagcttggagcgaacgacctacaccgaactgagatacctacagcgtgagcattgagaaagcgccacgcttcccgaagggagaaaggcggacaggtatccggtaagcggcagggtcggaacaggagagcgcacgagggagcttccagggggaaacgcctggtatctttatagtcctgtcgggtttcgccacctctgacttgagcgtcgatttttgtgatgctcgtcaggggggcggagcctatggaaaaacgccagcaacgcggcctttttacggttcctggccttttgctggccttttgctcacatgttctttcctgcgttatcccctgattctgtggataaccgtattaccgcctttgagtgagctgataccgctcgccgcagccgaacgaccgagcgcagcgagtcagtgagcgaggaagcggaagagcgcccaatacgcaaaccgcctctccccgcgcgttggccgattcattaatgcagctggcacgacaggtttcccgactggaaagcgggcagtgagcgcaacgcaattaatgtgagttagctcactcattaggcaccccaggctttacactttatgcttccggctcgtatgttgtgtggaattgtgagcggataacaatttcacacaggaaacagctatgaccatgattacgccaagctttgctcttaggagtttcctaatacatcccaaactcaaatatataaagcatttgacttgttctatgccctagggggcggggggaagctaagccagctttttttaacatttaaaatgttaattccattttaaatgcacagatgtttttatttcataagggtttcaatgtgcatgaatgctgcaatattcctgttaccaaagctagtataaataaaaatagataaacgtggaaattacttagagtttctgtcattaacgtttccttcctcagttgacaacataaatgcgctgctgagcaagccagtttgcatctgtcaggatcaatttcccattatgccagtcatattaattactagtcaattagttgatttttatttttgacatatacatgtgaatgaaagaccccacctgtaggtttggcaagctagcttaagtaacgccattttgcaaggcatggaaaaatacataactgagaatagaaaagttcagatcaaggtcaggaacagatggaacagctgaatatgggccaaacaggatatctgtggtaagcagttcctgccccggctcagggccaagaacagatggaacagctgaatatgggccaaacaggatatctgtggtaagcagttcctgccccggctcagggccaagaacagatggtccccagatgcggtccagccctcagcagtttctagagaaccatcagatgtttccagggtgccccaaggacctgaaatgaccctgtgccttatttgaactaaccaatcagttcgcttctcgcttctgttcgcgcgcttatgctccccgagctcaataaaagagcccacaacccctcactcggggcgccagtcctccgattgactgagtcgcccgggtacccgtgtatccaataaaccctcttgcagttgcatccgacttgtggtctcgctgttccttgggagggtctcctctgagtgattgactacccgtcagcgggggtctttcatttgggggctcgtccgggatcgggagacccctgcccagggaccaccgacccaccaccgggaggtaagctggccagcaacttatctgtgtctgtccgattgtctagtgtctatgactgattttatgcgcctgcgtcggtactagttagctaactagctctgtatctggcggacccgtggtggaactgacgagttcggaacacccggccgcaaccctgggagacgtcccagggacttcgggggccgtttttgtggcccgacctgagtcctaaaatcccgatcgtttaggactctttggtgcaccccccttagaggagggatatgtggttctggtaggagacgagaacctaaaacagttcccgcctccgtctgaatttttgctttcggtttgggaccgaagccgcgccgcgcgtcttgtctgctgcagcatcgttctgtgttgtctctgtctgactgtgtttctgtatttgtctgaaaatatgggcccgggctagactgttaccactcccttaagtttgaccttaggtcactggaaagatgtcgagcggatcgctcacaaccagtcggtagatgtcaagaagagacgttgggttaccttctgctctgcagaatggccaacctttaacgtcggatggccgcgagacggcacctttaaccgagacctcatcacccaggttaagatcaaggtcttttcacctggcccgcatggacacccagaccaggtcccctacatcgtgacctgggaagccttggcttttgacccccctccctgggtcaagccctttgtacaccctaagcctccgcctcctcttcctccatccgccccgtctctcccccttgaacctcctcgttcgaccccgcctcgatcctccctttatccagccctcact

SEQ ID NO: 233 - DNA, 7641 bp, synthetic construct
  misc_feature 1..7641: note = Description of Artificial Sequence: Synthetic polynucleotide
  source 1..7641: mol_type = other DNA
ccttctctaggcgcccccatatggccatatgagatcttatatggggcacccccgccccttgtaaacttccctgaccctgacatgacaagagttactaacagcccctctctccaagctcacttacaggctctctacttagtccagcacgaagtctggagacctctggcggcagcctaccaagaacaactggaccgaccggtgccgccaccatggaaaccgacaccctgctgctgtgggtgctgctgctgtgggtgccaggatccacaggacaatctgccctgactcagcctgcctccgtgtctgcgtctcctggacagtcgatcgccatctcctgcactggaaccagcagtgacgttggttggtatcaacagcacccaggcaaagcccccaaactcatgatttatgaggacagtaagcggccctcaggggtttctaatcgcttctctggctccaagtctggcaacacggcctccctgaccatctctgggctccaggctgaggacgaggctgattattactgcagctcaaatacaagaagcagcactttggtgttcggcggagggaccaagctgaccgtcctaggttctagaggtggtggtggtagcggcggcggcggctctggtggtggtggatccctcgagatggccgaagtgcagctggtgcagtctggggctgagatgaagaagcctggggcctcactgaagctctcctgcaaggcttctggatacaccttcatcgactactatgtatactggatgcgacaggcccctggacaagggcttgagtccatgggatggatcaaccctaacagtggtggcacaaactatgcacagaagtttcagggcagggtcaccatgaccagggacacgtccatcagcacagcctacatggagctgagcaggctgagatctgacgacaccgccatgtattactgtgcgcgctcccagcgtgacggttacatggattactggggtcaaggtactctggtgaccgtctcctcagcggccgcacccaccacgacgccagcgccgcgaccaccaaccccggcgcccacgatcgcgtcgcagcccctgtccctgcgcccagaggcgtgccggccagcggcggggggcgcagtgcacacgagggggctggacttcgcctgtgatatctacatctgggcgcccctggccgggacttgtggggtccttctcctgtcactggttatcaccctttactgcaacaaacggggcagaaagaagctcctgtatatattcaaacaaccatttatgagaccagtacaaactactcaagaggaagatggctgtagctgccgatttccagaagaagaagaaggaggatgtgaactgagagtgaagttcagcaggagcgcagagccccccgcgtaccagcagggccagaaccagctctataacgagctcaatctaggacgaagagaggagtacgatgttttggacaagagacgtggccgggaccctgagatggggggaaagccgagaaggaagaaccctcaggaaggcctgtacaatgaactgcagaaagataagatggcggaggcctacagtgagattgggatgaaaggcgagcgccggaggggcaaggggcacgatggcctttaccagggtctcagtacagccaccaaggacacctacgacgcccttcacatgcaggccctgccccctcgctaacagccactcgaggatccggattagtccaatttgttaaagacaggatatcagtggtccaggctctagttttgactcaacaatatcaccagctgaagcctatagagtacgagccatagataaaataaaagattttatttagtctccagaaaaaggggggaatgaaagaccccacctgtaggtttggcaagctagcttaagtaacgccattttgcaaggcatggaaaaatacataactgagaatagagaagttcagatcaaggtcaggaacagatggaacagctgaatatgggccaaacaggatatctgtggtaagcagttcctgccccggctcagggccaagaacagatggaacagctgaatatgggccaaacaggatatctgtggtaagcagttcctgccccggctcagggccaagaacagatggtccccagatgcggtccagccctcagcagtttctagagaaccatcagatgtttccagggtgccccaaggacctgaaatgaccctgtgccttatttgaactaaccaatcagttcgcttctcgcttctgttcgcgcgcttctgctccccgagctcaataaaagagcccacaacccctcactcggggcgccagtcctccgattgactgagtcgcccgggtacccgtgtatccaataaaccctcttgcagttgcatccgacttgtggtctcgctgttccttgggagggtctcctctgagtgattgactacccgtcagcgggggtctttcacacatgcagcatgtatcaaaattaatttggttttttttcttaagtatttacattaaatggccatagtacttaaagttacattggcttccttgaaataaacatggagtattcagaatgtgtcataaatatttctaattttaagatagtatctccattggctttctactttttcttttatttttttttgtcctctgtcttccatttgttgttgttgttgtttgtttgtttgtttgttggttggttggttaatttttttttaaagatcctacactatagttcaagctagactattagctactctgtaacccagggtgaccttgaagtcatgggtagcctgctgttttagccttcccacatctaagattacaggtatgagctatcatttttggtatattgattgattgattgattgatgtgtgtgtgtgtgattgtgtttgtgtgtgtgactgtgaaaatgtgtgtatgggtgtgtgtgaatgtgtgtatgtatgtgtgtgtgtgagtgtgtgtgtgtgtgtgtgcatgtgtgtgtgtgtgactgtgtctatgtgtatgactgtgtgtgtgtgtgtgtgtgtgtgtgtgtgtgtgtgtgtgtgtgtgttgtgaaaaaatattctatggtagtgagagccaacgctccggctcaggtgtcaggttggtttttgagacagagtctttcacttagcttggaattcactggccgtcgttttacaacgtcgtgactgggaaaaccctggcgttacccaacttaatcgccttgcagcacatccccctttcgccagctggcgtaatagcgaagaggcccgcaccgatcgcccttcccaacagttgcgcagcctgaatggcgaatggcgcctgatgcggtattttctccttacgcatctgtgcggtatttcacaccgcatatggtgcactctcagtacaatctgctctgatgccgcatagttaagccagccccgacacccgccaacacccgctgacgcgccctgacgggcttgtctgctcccggcatccgcttacagacaagctgtgaccgtctccgggagctgcatgtgtcagaggttttcaccgtcatcaccgaaacgcgcgatgacgaaagggcctcgtgatacgcctatttttataggttaatgtcatgataataatggtttcttagacgtcaggtggcacttttcggggaaatgtgcgcggaacccctatttgtttatttttctaaatacattcaaatatgtatccgctcatgagacaataaccctgataaatgcttcaataatattgaaaaaggaagagtatgagtattcaacatttccgtgtcgcccttattcccttttttgcggcattttgccttcctgtttttgctcacccagaaacgctggtgaaagtaaaagatgctgaagatcagttgggtgcacgagtgggttacatcgaactggatctcaacagcggtaagatccttgagagttttcgccccgaagaacgttttccaatgatgagcacttttaaagttctgctatgtggcgcggtattatcccgtattgacgccgggcaagagcaactcggtcgccgcatacactattctcagaatgacttggttgagtactcaccagtcacagaaaagcatcttacggatggcatgacagtaagagaattatgcagtgctgccataaccatgagtgataacactgcggccaacttacttctgacaacgatcggaggaccgaaggagctaaccgcttttttgcacaacatgggggatcatgtaactcgccttgatcgttgggaaccggagctgaatgaagccataccaaacgacgagcgtgacaccacgatgcctgtagcaatggcaacaacgttgcgcaaactattaactggcgaactacttactctagcttcccggcaacaattaatagactggatggaggcggataaagttgcaggaccacttctgcgctcggcccttccggctggctggtttattgctgataaatctggagccggtgagcgtgggtctcgcggtatcattgcagcactggggccagatggtaagccctcccgtatcgtagttatctacacgacggggagtcaggcaactatggatgaacgaaatagacagatcgctgagataggtgcctcactgattaagcattggtaactgtcagaccaagtttactcatatatactttagattgatttaaaacttcatttttaatttaaaaggatctaggtgaagatcctttttgataatctcatgaccaaaatcccttaacgtgagttttcgttccactgagcgtcagaccccgtagaaaagatcaaaggatcttcttgagatcctttttttctgcgcgtaatctgctgcttgcaaacaaaaaaaccaccgctaccagcggtggtttgtttgccggatcaagagctaccaactctttttccgaaggtaactggcttcagcagagcgcagataccaaatactgtccttctagtgtagccgtagttaggccaccacttcaagaactctgtagcaccgcctacatacctcgctctgctaatcctgttaccagtggctgctgccagtggcgataagtcgtgtcttaccgggttggactcaagacgatagttaccggataaggcgcagcggtcgggctgaacggggggttcgtgcacacagcccagcttggagcgaacgacctacaccgaactgagatacctacagcgtgagcattgagaaagcgccacgcttcccgaagggagaaaggcggacaggtatccggtaagcggcagggtcggaacaggagagcgcacgagggagcttccagggggaaacgcctggtatctttatagtcctgtcgggtttcgccacctctgacttgagcgtcgatttttgtgatgctcgtcaggggggcggagcctatggaaaaacgccagcaacgcggcctttttacggttcctggccttttgctggccttttgctcacatgttctttcctgcgttatcccctgattctgtggataaccgtattaccgcctttgagtgagctgataccgctcgccgcagccgaacgaccgagcgcagcgagtcagtgagcgaggaagcggaagagcgcccaatacgcaaaccgcctctccccgcgcgttggccgattcattaatgcagctggcacgacaggtttcccgactggaaagcgggcagtgagcgcaacgcaattaatgtgagttagctcactcattaggcaccccaggctttacactttatgcttccggctcgtatgttgtgtggaattgtgagcggataacaatttcacacaggaaacagctatgaccatgattacgccaagctttgctcttaggagtttcctaatacatcccaaactcaaatatataaagcatttgacttgttctatgccctagggggcggggggaagctaagccagctttttttaacatttaaaatgttaattccattttaaatgcacagatgtttttatttcataagggtttcaatgtgcatgaatgctgcaatattcctgttaccaaagctagtataaataaaaatagataaacgtggaaattacttagagtttctgtcattaacgtttccttcctcagttgacaacataaatgcgctgctgagcaagccagtttgcatctgtcaggatcaatttcccattatgccagtcatattaattactagtcaattagttgatttttatttttgacatatacatgtgaatgaaagaccccacctgtaggtttggcaagctagcttaagtaacgccattttgcaaggcatggaaaaatacataactgagaatagaaaagttcagatcaaggtcaggaacagatggaacagctgaatatgggccaaacaggatatctgtggtaagcagttcctgccccggctcagggccaagaacagatggaacagctgaatatgggccaaacaggatatctgtggtaagcagttcctgccccggctcagggccaagaacagatggtccccagatgcggtccagccctcagcagtttctagagaaccatcagatgtttccagggtgccccaaggacctgaaatgaccctgtgccttatttgaactaaccaatcagttcgcttctcgcttctgttcgcgcgcttatgctccccgagctcaataaaagagcccacaacccctcactcggggcgccagtcctccgattgactgagtcgcccgggtacccgtgtatccaataaaccctcttgcagttgcatccgacttgtggtctcgctgttccttgggagggtctcctctgagtgattgactacccgtcagcgggggtctttcatttgggggctcgtccgggatcgggagacccctgcccagggaccaccgacccaccaccgggaggtaagctggccagcaacttatctgtgtctgtccgattgtctagtgtctatgactgattttatgcgcctgcgtcggtactagttagctaactagctctgtatctggcggacccgtggtggaactgacgagttcggaacacccggccgcaaccctgggagacgtcccagggacttcgggggccgtttttgtggcccgacctgagtcctaaaatcccgatcgtttaggactctttggtgcaccccccttagaggagggatatgtggttctggtaggagacgagaacctaaaacagttcccgcctccgtctgaatttttgctttcggtttgggaccgaagccgcgccgcgcgtcttgtctgctgcagcatcgttctgtgttgtctctgtctgactgtgtttctgtatttgtctgaaaatatgggcccgggctagactgttaccactcccttaagtttgaccttaggtcactggaaagatgtcgagcggatcgctcacaaccagtcggtagatgtcaagaagagacgttgggttaccttctgctctgcagaatggccaacctttaacgtcggatggccgcgagacggcacctttaaccgagacctcatcacccaggttaagatcaaggtcttttcacctggcccgcatggacacccagaccaggtcccctacatcgtgacctgggaagccttggcttttgacccccctccctgggtcaagccctttgtacaccctaagcctccgcctcctcttcctccatccgccccgtctctcccccttgaacctcctcgttcgaccccgcctcgatcctccctttatccagccctcact

SEQ ID NO: 234 - DNA, 1491 bp, synthetic construct
  misc_feature 1..1491: note = Description of Artificial Sequence: Synthetic polynucleotide
  source 1..1491: mol_type = other DNA
atggaaaccgacaccctgctgctgtgggtgctgctgctgtgggtgccaggatccacaggactgcctgtgctgactcagccaccctcagcgtctgggacccccgggcagagggtcaccatctcttgttctggacgcagttccaacatcgggagtaattctgttaactggtatcgacaactcccaggagcggcccccaaactcctcatctatagtaataatcagcggcccccaggggtccctgtgcgattctctggctccaagtctggcacctcagcctccctggccatcagtgggctccagtctgaagatgaggccacttattactgtgcaacatgggatgacaatctgaatgttcactatgtcttcggaactgggaccaaggtcaccgtcctaggttctagaggtggtggtggtagcggcggcggcggctctggtggtggtggatccctcgagatggcccaggtgcagctggtgcagtctggggctgaggtgaagaagcctgggtcctcggtgaaggtctcctgcaaggcttctggaggcaccttcagcagctatgctatcagctgggtgcgacaggcccctggacaagggcttgagtggatgggaaggatcatccctatccttggtatagcaaactacgcacagaagttccagggcagagtcacgattaccgcggacaaatccacgagcacagcctacatggagctgagcagcctgagatctgaggacacggccgtgtattactgtgcgcgcggtggttactactctcatgacatgtggtctgaagattggggtcaaggtactctggtgaccgtctcctcagcggccgcaattgaagttatgtatcctcctccttacctagacaatgagaagagcaatggaaccattatccatgtgaaagggaaacacctttgtccaagtcccctatttcccggaccttctaagcccttttgggtgctggtggtggttggtggagtcctggcttgctatagcttgctagtaacagtggcctttattattttctgggtgaggagtaagaggagcaggctcctgcacagtgactacatgaacatgactccccgccgccccgggcccacccgcaagcattaccagccctatgccccaccacgcgacttcgcagcctatcgctccagagtgaagttcagcaggagcgcagacgcccccgcgtaccagcagggccagaaccagctctataacgagctcaatctaggacgaagagaggagtacgatgttttggacaagagacgtggccgggaccctgagatggggggaaagccgagaaggaagaaccctcaggaaggcctgtacaatgaactgcagaaagataagatggcggaggcctacagtgagattgggatgaaaggcgagcgccggaggggcaaggggcacgatggcctttaccagggtctcagtacagccaccaaggacacctacgacgcccttcacatgcaggccctgccccctcgctaa

SEQ ID NO: 235 - DNA, 1488 bp, synthetic construct
  misc_feature 1..1488: note = Description of Artificial Sequence: Synthetic polynucleotide
  source 1..1488: mol_type = other DNA
atggaaaccgacaccctgctgctgtgggtgctgctgctgtgggtgccaggatccacaggacaggctgtgctgactcagccaccctcagcgtctgggacccccgggcagagggtcaccatctcttgttctggaagcagctccaacatcggaagtaattacgtattctggtaccagcagctcccaggaacggcccccaaactcctcatctatagtaataatcagcggccctcaggggtccctgaccgattctctggctccaagtctggcacctcagcctccctggccatcagtgggctccggtccgaggatgaggctgattattactgtgcagcatgggatgacagcctgagtgcctcttatgttttcggaactgggaccaaggtcaccgtcctaggttctagaggtggtggtggtagcggcggcggcggctctggtggtggtggatccctcgagatggcccaggtgcagctggtgcagtctggggctgaggtgaagaagcctgggtcctcggtgaaggtctcctgcaaggcttctggaggcaccttcagcagctatgctatcagctgggtgcgacaggcccctggacaagggcttgagtggatgggaaggatcatccctatccttggtacagcaaactacgcacagaagttccagggcagagtcacgattaccgcggacgaatccacgagcacagcctacatggagctgagcagcctgagatctgaggacacggccgtgtattactgtgcgcgctctggttacggttcttaccgttgggaagattcttggggtcaaggtactctggtgaccgtctcctcagcggccgcaattgaagttatgtatcctcctccttacctagacaatgagaagagcaatggaaccattatccatgtgaaagggaaacacctttgtccaagtcccctatttcccggaccttctaagcccttttgggtgctggtggtggttggtggagtcctggcttgctatagcttgctagtaacagtggcctttattattttctgggtgaggagtaagaggagcaggctcctgcacagtgactacatgaacatgactccccgccgccccgggcccacccgcaagcattaccagccctatgccccaccacgcgacttcgcagcctatcgctccagagtgaagttcagcaggagcgcagacgcccccgcgtaccagcagggccagaaccagctctataacgagctcaatctaggacgaagagaggagtacgatgttttggacaagagacgtggccgggaccctgagatggggggaaagccgagaaggaagaaccctcaggaaggcctgtacaatgaactgcagaaagataagatggcggaggcctacagtgagattgggatgaaaggcgagcgccggaggggcaaggggcacgatggcctttaccagggtctcagtacagccaccaaggacacctacgacgcccttcacatgcaggccctgccccctcgctaa

SEQ ID NO: 236 - protein, 19 aa, synthetic construct
  REGION 1..19: note = Description of Artificial Sequence: Synthetic peptide
SGSGLQMAGQCSQNEYFDS

SEQ ID NO: 237 - protein, 19 aa, synthetic construct
  REGION 1..19: note = Description of Artificial Sequence: Synthetic peptide
SGSGQMAGQCSQNEYFDSL

SEQ ID NO: 238 - protein, 19 aa, synthetic construct
  REGION 1..19: note = Description of Artificial Sequence: Synthetic peptide
SGSGMAGQCSQNEYFDSLL

SEQ ID NO: 239 - protein, 19 aa, synthetic construct
  REGION 1..19: note = Description of Artificial Sequence: Synthetic peptide
SGSGAGQCSQNEYFDSLLH

SEQ ID NO: 240 - protein, 19 aa, synthetic construct
  REGION 1..19: note = Description of Artificial Sequence: Synthetic peptide
SGSGGQCSQNEYFDSLLHA

SEQ ID NO: 241 - protein, 19 aa, synthetic construct
  REGION 1..19: note = Description of Artificial Sequence: Synthetic peptide
SGSGQCSQNEYFDSLLHAC

SEQ ID NO: 242 - protein, 19 aa, synthetic construct
  REGION 1..19: note = Description of Artificial Sequence: Synthetic peptide
SGSGCSQNEYFDSLLHACI

SEQ ID NO: 243 - protein, 19 aa, synthetic construct
  REGION 1..19: note = Description of Artificial Sequence: Synthetic peptide
SGSGSQNEYFDSLLHACIP

SEQ ID NO: 244 - protein, 19 aa, synthetic construct
  REGION 1..19: note = Description of Artificial Sequence: Synthetic peptide
SGSGQNEYFDSLLHACIPC

SEQ ID NO: 245 - protein, 19 aa, synthetic construct
  REGION 1..19: note = Description of Artificial Sequence: Synthetic peptide
SGSGNEYFDSLLHACIPCQ

SEQ ID NO: 246 - protein, 19 aa, synthetic construct
  REGION 1..19: note = Description of Artificial Sequence: Synthetic peptide
SGSGEYFDSLLHACIPCQL

SEQ ID NO: 247 - protein, 19 aa, synthetic construct
  REGION 1..19: note = Description of Artificial Sequence: Synthetic peptide
SGSGYFDSLLHACIPCQLR

SEQ ID NO: 248 - protein, 19 aa, synthetic construct
  REGION 1..19: note = Description of Artificial Sequence: Synthetic peptide
SGSGFDSLLHACIPCQLRC

SEQ ID NO: 249 - protein, 19 aa, synthetic construct
  REGION 1..19: note = Description of Artificial Sequence: Synthetic peptide
SGSGDSLLHACIPCQLRCS

SEQ ID NO: 250 - protein, 19 aa, synthetic construct
  REGION 1..19: note = Description of Artificial Sequence: Synthetic peptide
SGSGSLLHACIPCQLRCSS

SEQ ID NO: 251 - protein, 19 aa, synthetic construct
  REGION 1..19: note = Description of Artificial Sequence: Synthetic peptide
SGSGLLHACIPCQLRCSSN

SEQ ID NO: 252 - protein, 19 aa, synthetic construct
  REGION 1..19: note = Description of Artificial Sequence: Synthetic peptide
SGSGLHACIPCQLRCSSNT

SEQ ID NO: 253 - protein, 19 aa, synthetic construct
  REGION 1..19: note = Description of Artificial Sequence: Synthetic peptide
SGSGHACIPCQLRCSSNTP

SEQ ID NO: 254 - protein, 19 aa, synthetic construct
  REGION 1..19: note = Description of Artificial Sequence: Synthetic peptide
SGSGACIPCQLRCSSNTPP

SEQ ID NO: 255 - protein, 19 aa, synthetic construct
  REGION 1..19: note = Description of Artificial Sequence: Synthetic peptide
SGSGCIPCQLRCSSNTPPL

SEQ ID NO: 256 - protein, 19 aa, synthetic construct
  REGION 1..19: note = Description of Artificial Sequence: Synthetic peptide
SGSGIPCQLRCSSNTPPLT

SEQ ID NO: 257 - protein, 19 aa, synthetic construct
  REGION 1..19: note = Description of Artificial Sequence: Synthetic peptide
SGSGPCQLRCSSNTPPLTC

SEQ ID NO: 258 - protein, 19 aa, synthetic construct
  REGION 1..19: note = Description of Artificial Sequence: Synthetic peptide
SGSGCQLRCSSNTPPLTCQ

SEQ ID NO: 259 - protein, 19 aa, synthetic construct
  REGION 1..19: note = Description of Artificial Sequence: Synthetic peptide
SGSGQLRCSSNTPPLTCQR

SEQ ID NO: 260 - protein, 19 aa, synthetic construct
  REGION 1..19: note = Description of Artificial Sequence: Synthetic peptide
SGSGLRCSSNTPPLTCQRY

SEQ ID NO: 261 - protein, 19 aa, synthetic construct
  REGION 1..19: note = Description of Artificial Sequence: Synthetic peptide
SGSGRCSSNTPPLTCQRYC

SEQ ID NO: 262 - protein, 19 aa, synthetic construct
  REGION 1..19: note = Description of Artificial Sequence: Synthetic peptide
SGSGCSSNTPPLTCQRYCN

SEQ ID NO: 263 - protein, 19 aa, synthetic construct
  REGION 1..19: note = Description of Artificial Sequence: Synthetic peptide
SGSGSSNTPPLTCQRYCNA

SEQ ID NO: 264 - protein, 19 aa, synthetic construct
  REGION 1..19: note = Description of Artificial Sequence: Synthetic peptide
SGSGSNTPPLTCQRYCNAS

SEQ ID NO: 265 - protein, 19 aa, synthetic construct
  REGION 1..19: note = Description of Artificial Sequence: Synthetic peptide
SGSGNTPPLTCQRYCNASV

SEQ ID NO: 266 - protein, 19 aa, synthetic construct
  REGION 1..19: note = Description of Artificial Sequence: Synthetic peptide
SGSGTPPLTCQRYCNASVT

SEQ ID NO: 267 - protein, 19 aa, synthetic construct
  REGION 1..19: note = Description of Artificial Sequence: Synthetic peptide
SGSGPPLTCQRYCNASVTN

SEQ ID NO: 268 - protein, 19 aa, synthetic construct
  REGION 1..19: note = Description of Artificial Sequence: Synthetic peptide
SGSGPLTCQRYCNASVTNS

SEQ ID NO: 269 - protein, 19 aa, synthetic construct
  REGION 1..19: note = Description of Artificial Sequence: Synthetic peptide
SGSGLTCQRYCNASVTNSV

SEQ ID NO: 270 - protein, 19 aa, synthetic construct
  REGION 1..19: note = Description of Artificial Sequence: Synthetic peptide
SGSGTCQRYCNASVTNSVK

SEQ ID NO: 271 - protein, 19 aa, synthetic construct
  REGION 1..19: note = Description of Artificial Sequence: Synthetic peptide
SGSGCQRYCNASVTNSVKG

SEQ ID NO: 272 - protein, 19 aa, synthetic construct
  REGION 1..19: note = Description of Artificial Sequence: Synthetic peptide
SGSGQRYCNASVTNSVKGT

SEQ ID NO: 273 - protein, 19 aa, synthetic construct
  REGION 1..19: note = Description of Artificial Sequence: Synthetic peptide
SGSGRYCNASVTNSVKGTN

SEQ ID NO: 274 - protein, 19 aa, synthetic construct
  REGION 1..19: note = Description of Artificial Sequence: Synthetic peptide
SGSGYCNASVTNSVKGTNA

SEQ ID NO: 275 - protein, 25 aa, synthetic construct
  REGION 1..25: note = Description of Artificial Sequence: Synthetic peptide
TSGQAGQHHHHHHGAYPYDVPDYAS

SEQ ID NO: 276 - DNA, 75 bp, synthetic construct
  misc_feature 1..75: note = Description of Artificial Sequence: Synthetic oligonucleotide
  source 1..75: mol_type = other DNA
actagtggccaggccggccagcaccatcaccatcaccatggcgcatacccgtacgacgttccggactacgcttct

SEQ ID NO: 277 - protein, 4 aa, Homo sapiens
YVKM

SEQ ID NO: 278 - protein, 4 aa, synthetic construct
  REGION 1..4: note = Description of Artificial Sequence: Synthetic peptide
SGSG

SEQ ID NO: 279 - protein, 5 aa, synthetic construct
  REGION 1..5: note = Description of Artificial Sequence: Synthetic peptide
GSSSS

SEQ ID NO: 280 - protein, 53 aa, synthetic construct
  REGION 1..53: note = Description of Artificial Sequence: Synthetic polypeptide
LQMAGQCSQNEYFDSLLHACIPCQLRCSSNTPPLTCQRYCNASVTNSVKGTNA